European Patent Application EP 4 464 779 A2, published November 20, 2024. Title: Pan-Genotype Agents Against Respiratory Viruses and Methods of Using the Same. Applicant: THE BOARD OF TRUSTEES OF THE LELAND STANFORD JUNIOR UNIVERSITY. Application EP. The sequence listing filed with the application follows.

SEQUENCE LISTING (908 sequences)

SEQ ID NO: 1 - RNA, 196 nt, synthetic construct
  misc_feature 1..196: note = Synthetic polynucleotide
  source 1..196: mol_type = other RNA
agtagaaacaaggtcgtttttaaactattcgacactaattgatggccatccgaattcttttggtcgctgtctggctgtcagtaagtatgctagagtcccgttttcgtttcattaccaacaccacgtctccttgcccaattagcacattagccttttttattctttccatattgaatataattgacctgctttcgct

SEQ ID NO: 2 - RNA, 182 nt, synthetic construct
  misc_feature 1..182: note = Synthetic polynucleotide
  source 1..182: mol_type = other RNA
agtagaaacaaggtcgtttttaaactattcgacactaattgatcgccatccgaattcttttggtcgctgtctggctgtcagtaagtatgctagagtcccgttttcgtttcgcgagactgcgacattagatttcttagttcttttattctttccatattgaatataattgacctgctttcgct

SEQ ID NO: 3 - RNA, 198 nt, synthetic construct
  misc_feature 1..198: note = Synthetic polynucleotide
  source 1..198: mol_type = other RNA
agtagaaacaaggtcgtttttaaactattcgacactaattgatggccatccgaattcttttggtcgctgtctggctgtctgtaagtatgctagagtcccgttttcgtttcggactctcaaaaacgtgcgagactgcgacattagatttcttagttcttttattctttccatattgaatataattgacctgctttcgct

SEQ ID NO: 4 - RNA, 155 nt, synthetic construct
  misc_feature 1..155: note = Synthetic polynucleotide
  source 1..155: mol_type = other RNA
agtagaaacaaggtcgtttttaaactattcgacactaattgatggccatccgaattcttttggtcgctgtctggctgtcagtaagtatgctagagtcccgtttccgtttcattaccaacaccacgtctcttgaatataattgacctgctttcgct

SEQ ID NO: 5 - RNA, 178 nt, synthetic construct
  misc_feature 1..178: note = Synthetic polynucleotide
  source 1..178: mol_type = other RNA
agtagaaacaaggtcgtttttaaataattcgacactaattgatggccatccgaattcttttggtcgctgtctggctgtcagtaagtatgctagagtcccgttttcgtttcattaccaacaccacgtctccttgcccttttattctctccatattgaatatatttgacctgctttcgct

SEQ ID NO: 6 - RNA, 290 nt, synthetic construct
  misc_feature 1..290: note = Synthetic polynucleotide
  source 1..290: mol_type = other RNA
agtagaaacaaggtcgtttttaaactattcgacactaattgatggccatccgaattcttttggtcgctgtctggctgtcagtaagtatgctagagtcccgttttcgtttcattaccaacactacgtccccttgcccaattagcacattagccttctctccttttgcaagattgctcagttcattgatgcttaatgctgggccatatctcttgtcttctttgcccaaaatgagaaatcctctcaggacagcatattctctccatattgaatataattgacctgctttcgct

SEQ ID NO: 7 - RNA, 178 nt, synthetic construct
  misc_feature 1..178: note = Synthetic polynucleotide
  modified_base 104: mod_base = i
  source 1..178: mol_type = other RNA
agtagaaacaaggtcgtttttaaactattcgacactaattgatggccatccgaattcttttggtcgctgtctggctgtcagtaagtatgctagagtcccgtttacgtttcattaccaacaccacgtctccttgcccttttattctttccatattgaatataattgacctgctttcgct

SEQ ID NO: 8 - RNA, 197 nt, synthetic construct
  misc_feature 1..197: note = Synthetic polynucleotide
  source 1..197: mol_type = other RNA
agtagaaacaaggtcgtttttaaactattcgacactaattgatggccatccgaattcttttggtcgctgtctggctgtcagttaatatgctagagtcccgttttcgtttcattaccaacaccacgtctccttgcccaattagcacgtcgataggttttttattctttccatattgaatataatgacctgctttcgct

SEQ ID NO: 9 - RNA, 198 nt, synthetic construct; identical to SEQ ID NO: 3
  misc_feature 1..198: note = Synthetic polynucleotide
  source 1..198: mol_type = other RNA

SEQ ID NO: 10 - RNA, 178 nt, synthetic construct
  misc_feature 1..178: note = Synthetic polynucleotide
  source 1..178: mol_type = other RNA
agtagaaacaaggtcgtttttaaactattcgacatctaattgatggccatccgaattcttttggtcgctgtctggctgtcagtaagtatgctagagtcccgttttcgtttgactgcgacattagatttcttagttcttttattctttccatattgaatataattgacctgctttcgct

SEQ ID NO: 11 - RNA, 182 nt, synthetic construct; identical to SEQ ID NO: 2
  misc_feature 1..182: note = Synthetic polynucleotide
  source 1..182: mol_type = other RNA

SEQ ID NO: 12 - RNA, 59 nt, synthetic construct
  misc_feature 1..59: note = Synthetic polynucleotide
  source 1..59: mol_type = other RNA
cgacactaattgatggccatccgaattcttttggtcgctgtctggctgtcagtaagtat

SEQ ID NO: 13 - RNA, 59 nt, synthetic construct; identical to SEQ ID NO: 12
  misc_feature 1..59: note = Synthetic polynucleotide
  source 1..59: mol_type = other RNA

SEQ ID NO: 14 - DNA, 108 bp, synthetic construct
  misc_feature 1..108: note = Synthetic polynucleotide
  source 1..108: mol_type = other DNA
attgggcaaggagacgtggtgttggtaatgaaacggaaacggaactctagcatacttactgacagccagacagcgaccaaaagaattcggatggccatcaattagtgt

SEQ ID NO: 15 - DNA, 108 bp, synthetic construct
  misc_feature 1..108: note = Synthetic polynucleotide
  source 1..108: mol_type = other DNA
attgggcaaggagacgtcgtgttggtaatgaaacggaaacggaactctagcatattaacagacagccaaacagcgacgaaaagaattcggatggcgatcaattgatgt

SEQ ID NO: 16 - DNA, 23 bp, synthetic construct
  misc_feature 1..23: note = Synthetic polynucleotide
  source 1..23: mol_type = other DNA
tacttactgacagtcagacagcg

SEQ ID NO: 17 - DNA, 23 bp, synthetic construct
  misc_feature 1..23: note = Synthetic polynucleotide
  source 1..23: mol_type = other DNA
cgctgtctgactgtcagtaagta

SEQ ID NO: 18 - DNA, 23 bp, synthetic construct
  misc_feature 1..23: note = Synthetic polynucleotide
  source 1..23: mol_type = other DNA
tacttactgactcgcagacagcg

SEQ ID NO: 19 - DNA, 23 bp, synthetic construct
  misc_feature 1..23: note = Synthetic polynucleotide
  source 1..23: mol_type = other DNA
cgctgtctgcgagtcagtaagta

SEQ ID NO: 20 - DNA, 30 bp, synthetic construct
  misc_feature 1..30: note = Synthetic polynucleotide
  source 1..30: mol_type = other DNA
tgacagccagactgcgaccaaaagaattcg

SEQ ID NO: 21 - DNA, 30 bp, synthetic construct
  misc_feature 1..30: note = Synthetic polynucleotide
  source 1..30: mol_type = other DNA
cgaattcttttggtcgcagtctggctgtca

SEQ ID NO: 22 - DNA, 24 bp, synthetic construct
  misc_feature 1..24: note = Synthetic polynucleotide
  source 1..24: mol_type = other DNA
agcgaccaaaagcattcggatggc

SEQ ID NO: 23 - DNA, 24 bp, synthetic construct
  misc_feature 1..24: note = Synthetic polynucleotide
  source 1..24: mol_type = other DNA
gccatccgaatgcttttggtcgct

SEQ ID NO: 24 - RNA, 176 nt, synthetic construct
  misc_feature 1..176: note = Synthetic polynucleotide
  source 1..176: mol_type = other RNA
agtagaaacaaggtcgtttttaaactattcgacactaattgatggccatccgaattcttttggtcgctgtctggctgtcagtaagtatgctagagtcccgttttcgtttcattaccaacacgacgtctccttgcttttattctttccatattgaatataattgacctgctttcgct

SEQ ID NO: 25 - RNA, 151 nt, synthetic construct
  misc_feature 1..151: note = Synthetic polynucleotide
  source 1..151: mol_type = other RNA
agtagaaacaaggtcgtttttaaactattcgacactaattgatggccatccgaattcttttcgtcgctgtctggctgtcagtaagtatgctagagtcccgttttcgtttctttattctttccatattgaatataattgacctgctttcgct

SEQ ID NO: 26 - RNA, 149 nt, synthetic construct
  misc_feature 1..149: note = Synthetic polynucleotide
  source 1..149: mol_type = other RNA
agtagaaacaaggtcgtttttaaactattcgacactaattgatggccatccgaattcttttggtcgctgtttggctgtcagtaagtatgctagagtcccgttttagtttttattctttccatattgaatataattgacctgctttcgct

SEQ ID NO: 27 - RNA, 59 nt, synthetic construct; identical to SEQ ID NO: 12
  misc_feature 1..59: note = Synthetic polynucleotide
  source 1..59: mol_type = other RNA

SEQ ID NO: 28 - DNA, 29 bp, synthetic construct
  misc_feature 1..29: note = Synthetic polynucleotide
  source 1..29: mol_type = other DNA
agaattcggatgcccatcaattagtgtcg

SEQ ID NO: 29 - DNA, 29 bp, synthetic construct
  misc_feature 1..29: note = Synthetic polynucleotide
  source 1..29: mol_type = other DNA
cgacactaattgatgggcatccgaattct

SEQ ID NO: 30 - DNA, 23 bp, synthetic construct
  misc_feature 1..23: note = Synthetic polynucleotide
  source 1..23: mol_type = other DNA
tacttactgacaggcagacagcg

SEQ ID NO: 31 - DNA, 23 bp, synthetic construct
  misc_feature 1..23: note = Synthetic polynucleotide
  source 1..23: mol_type = other DNA
cgctgtctgcctgtcagtaagta

SEQ ID NO: 32 - DNA, 25 bp, synthetic construct
  misc_feature 1..25: note = Synthetic polynucleotide
  source 1..25: mol_type = other DNA
ttcggatgggcatcaattagtgtcg

SEQ ID NO: 33 - DNA, 25 bp, synthetic construct
  misc_feature 1..25: note = Synthetic polynucleotide
  source 1..25: mol_type = other DNA
cgacactaattgatgcccatccgaa

SEQ ID NO: 34 - DNA, 24 bp, synthetic construct
  misc_feature 1..24: note = Synthetic polynucleotide
  source 1..24: mol_type = other DNA
atacttactgacacccagacagcg

SEQ ID NO: 35 - DNA, 24 bp, synthetic construct
  misc_feature 1..24: note = Synthetic polynucleotide
  source 1..24: mol_type = other DNA
cgctgtctgggtgtcagtaagtat

SEQ ID NO: 36 - DNA, 24 bp, synthetic construct
  misc_feature 1..24: note = Synthetic polynucleotide
  source 1..24: mol_type = other DNA
tcggatggccatgaattagtgtcg

SEQ ID NO: 37 - DNA, 24 bp, synthetic construct
  misc_feature 1..24: note = Synthetic polynucleotide
  source 1..24: mol_type = other DNA
cgacactaattcatggccatccga

SEQ ID NO: 38 - DNA, 26 bp, synthetic construct
  misc_feature 1..26: note = Synthetic polynucleotide
  source 1..26: mol_type = other DNA
agcatacttactcacagccagacagc

SEQ ID NO: 39 - DNA, 26 bp, synthetic construct
  misc_feature 1..26: note = Synthetic polynucleotide
  source 1..26: mol_type = other DNA
gctgtctggctgtgagtaagtatgct

SEQ ID NO: 40 - DNA, 34 bp, synthetic construct
  misc_feature 1..34: note = Synthetic polynucleotide
  source 1..34: mol_type = other DNA
ccaaaagaattaggatggccatcaattagtgtcg

SEQ ID NO: 41 - DNA, 34 bp, synthetic construct
  misc_feature 1..34: note = Synthetic polynucleotide
  source 1..34: mol_type = other DNA
cgacactaattgatggccatcctaattcttttgg

SEQ ID NO: 42 - DNA, 29 bp, synthetic construct
  misc_feature 1..29: note = Synthetic polynucleotide
  source 1..29: mol_type = other DNA
gacagccagacagctaccaaaagaattcg

SEQ ID NO: 43 - DNA, 29 bp, synthetic construct
  misc_feature 1..29: note = Synthetic polynucleotide
  source 1..29: mol_type = other DNA
cgaattcttttggtagctgtctggctgtc

SEQ ID NO: 44 - RNA, 71 nt, synthetic construct
  misc_feature 1..71: note = Synthetic polynucleotide
  source 1..71: mol_type = other RNA
tcgacactaattgatggccatccgaattcttttggtcgctgtctggctgtcagtaagtatgctagccttgc

SEQ ID NO: 45 - DNA, 11 bp, synthetic construct
  misc_feature 1..11: note = Synthetic polynucleotide
  source 1..11: mol_type = other DNA
accaaaagaat

SEQ ID NO: 46 - DNA, 11 bp, synthetic construct
  misc_feature 1..11: note = Synthetic polynucleotide
  source 1..11: mol_type = other DNA
tggccatcaat

SEQ ID NO: 47 - DNA, 11 bp, synthetic construct
  misc_feature 1..11: note = Synthetic polynucleotide
  source 1..11: mol_type = other DNA
tagcatactta

SEQ ID NO: 48-49 - skipped (2 entries)

SEQ ID NO: 50 - DNA, 15 bp, synthetic construct
  misc_feature 1..15: note = Synthetic polynucleotide
  source 1..15: mol_type = other DNA
cagacacgaccaaaa

SEQ ID NO: 51 - DNA, 15 bp, synthetic construct
  misc_feature 1..15: note = Synthetic polynucleotide
  source 1..15: mol_type = other DNA
tacttactgacagcc

SEQ ID NO: 52 - DNA, 15 bp, synthetic construct
  misc_feature 1..15: note = Synthetic polynucleotide
  source 1..15: mol_type = other DNA
agacacgaccaaaag

SEQ ID NO: 53 - DNA, 11 bp, synthetic construct
  misc_feature 1..11: note = Synthetic polynucleotide
  source 1..11: mol_type = other DNA
accaaaagaat

SEQ ID NO: 54 - DNA, 11 bp, synthetic construct
  misc_feature 1..11: note = Synthetic polynucleotide
  source 1..11: mol_type = other DNA
tggccatcaat

SEQ ID NO: 55 - DNA, 11 bp, synthetic construct
  misc_feature 1..11: note = Synthetic polynucleotide
  source 1..11: mol_type = other DNA
tagcatactta

SEQ ID NO: 56 - DNA, 15 bp, synthetic construct
  misc_feature 1..15: note = Synthetic polynucleotide
  source 1..15: mol_type = other DNA
cgaccaaaagaattc

SEQ ID NO: 57 - DNA, 15 bp, synthetic construct
  misc_feature 1..15: note = Synthetic polynucleotide
  source 1..15: mol_type = other DNA
cgaccaaaagaattc

SEQ ID NO: 58 - DNA, 15 bp, synthetic construct
  misc_feature 1..15: note = Synthetic polynucleotide
  source 1..15: mol_type = other DNA
gatggccatcaatta

SEQ ID NO: 59 - DNA, 15 bp, synthetic construct
  misc_feature 1..15: note = Synthetic polynucleotide
  source 1..15: mol_type = other DNA
gatggccatcaatta

SEQ ID NO: 60 - DNA, 15 bp, synthetic construct
  misc_feature 1..15: note = Synthetic polynucleotide
  source 1..15: mol_type = other DNA
tctagcatacttact

SEQ ID NO: 61 - DNA, 15 bp, synthetic construct
  misc_feature 1..15: note = Synthetic polynucleotide
  source 1..15: mol_type = other DNA
tctagcatacttact

SEQ ID NO: 62 - DNA, 15 bp, synthetic construct
  misc_feature 1..15: note = Synthetic polynucleotide
  source 1..15: mol_type = other DNA
gaattcggatggcca

SEQ ID NO: 63 - DNA, 15 bp, synthetic construct
  misc_feature 1..15: note = Synthetic polynucleotide
  source 1..15: mol_type = other DNA
ggccatcaattagtg

SEQ ID NO: 64 - DNA, 15 bp, synthetic construct
  misc_feature 1..15: note = Synthetic polynucleotide
  source 1..15: mol_type = other DNA
ttcggatggccatca

SEQ ID NO: 65 - DNA, 13 bp, synthetic construct
  misc_feature 1..13: note = Synthetic polynucleotide
  source 1..13: mol_type = other DNA
agccagacagcga

SEQ ID NO: 66 - DNA, 15 bp, synthetic construct
  misc_feature 1..15: note = Synthetic polynucleotide
  source 1..15: mol_type = other DNA
gacagccagacagca

SEQ ID NO: 67 - DNA, 11 bp, synthetic construct
  misc_feature 1..11: note = Synthetic polynucleotide
  misc_feature 1: note = LNA
  misc_feature 4: note = LNA
  misc_feature 7..8: note = LNA
  misc_feature 11: note = LNA
  source 1..11: mol_type = other DNA
accaaaagaat

SEQ ID NO: 68 - DNA, 11 bp, synthetic construct
  misc_feature 1..11: note = Synthetic polynucleotide
  misc_feature 1: note = LNA
  misc_feature 4: note = LNA
  misc_feature 6..7: note = LNA
  misc_feature 11: note = LNA
  source 1..11: mol_type = other DNA
tggccatcaat

SEQ ID NO: 69 - DNA, 11 bp, synthetic construct
  misc_feature 1..11: note = Synthetic polynucleotide
  misc_feature 1: note = LNA
  misc_feature 4..5: note = LNA
  misc_feature 7: note = LNA
  misc_feature 11: note = LNA
  source 1..11: mol_type = other DNA
tagcatactta

SEQ ID NO: 70-71 - skipped (2 entries)

SEQ ID NO: 72 - DNA, 15 bp, synthetic construct
  misc_feature 1..15: note = Synthetic polynucleotide
  misc_feature 1: note = LNA
  misc_feature 5: note = LNA
  misc_feature 7..8: note = LNA
  misc_feature 10..11: note = LNA
  misc_feature 14..15: note = LNA
  source 1..15: mol_type = other DNA
cagacacgaccaaaa

SEQ ID NO: 73 - DNA, 15 bp, synthetic construct
  misc_feature 1..15: note = Synthetic polynucleotide
  misc_feature 1..2: note = LNA
  misc_feature 4: note = LNA
  misc_feature 7..8: note = LNA
  misc_feature 11: note = LNA
  misc_feature 14..15: note = LNA
  source 1..15: mol_type = other DNA
tacttactgacagcc

SEQ ID NO: 74 - DNA, 15 bp, synthetic construct
  misc_feature 1..15: note = Synthetic polynucleotide
  misc_feature 1..4: note = LNA
  misc_feature 12..15: note = LNA
  source 1..15: mol_type = other DNA
agacacgaccaaaag

SEQ ID NO: 75 - DNA, 15 bp, synthetic construct
  misc_feature 1..15: note = Synthetic polynucleotide
  misc_feature 1..4: note = LNA
  misc_feature 13..15: note = LNA
  source 1..15: mol_type = other DNA
tacttactgacagcc

SEQ ID NO: 76 - DNA, 15 bp, synthetic construct
  misc_feature 1..15: note = Synthetic polynucleotide
  misc_feature 1..3: note = LNA
  misc_feature 12..15: note = LNA
  source 1..15: mol_type = other DNA
tacttactgacagcc

SEQ ID NO: 77 - DNA, 11 bp, synthetic construct
  misc_feature 1..11: note = Synthetic polynucleotide
  misc_feature 1..3: note = LNA
  misc_feature 9..11: note = LNA
  source 1..11: mol_type = other DNA
accaaaagaat

SEQ ID NO: 78 - DNA, 11 bp, synthetic construct
  misc_feature 1..11: note = Synthetic polynucleotide
  misc_feature 1..3: note = LNA
  misc_feature 9..11: note = LNA
  source 1..11: mol_type = other DNA
tggccatcaat

SEQ ID NO: 79 - DNA, 11 bp, synthetic construct
  misc_feature 1..11: note = Synthetic polynucleotide
  misc_feature 1..3: note = LNA
  misc_feature 9..11: note = LNA
  source 1..11: mol_type = other DNA
tagcatactta

SEQ ID NO: 80 - DNA, 15 bp, synthetic construct
  misc_feature 1..15: note = Synthetic polynucleotide
  misc_feature 1: note = LNA
  misc_feature 5..6: note = LNA
  misc_feature 9..10: note = LNA
  misc_feature 15: note = LNA
  source 1..15: mol_type = other DNA
cgaccaaaagaattc

SEQ ID NO: 81 - DNA, 15 bp, synthetic construct
  misc_feature 1..15: note = Synthetic polynucleotide
  misc_feature 1..4: note = LNA
  misc_feature 12..15: note = LNA
  source 1..15: mol_type = other DNA
cgaccaaaagaattc

SEQ ID NO: 82 - DNA, 15 bp, synthetic construct
  misc_feature 1..15: note = Synthetic polynucleotide
  misc_feature 1: note = LNA
  misc_feature 3..4: note = LNA
  misc_feature 6: note = LNA
  misc_feature 8..9: note = LNA
  misc_feature 12: note = LNA
  misc_feature 15: note = LNA
  source 1..15: mol_type = other DNA
gatggccatcaatta

SEQ ID NO: 83 - DNA, 15 bp, synthetic construct
  misc_feature 1..15: note = Synthetic polynucleotide
  misc_feature 1..4: note = LNA
  misc_feature 12..15: note = LNA
  source 1..15: mol_type = other DNA
gatggccatcaatta

SEQ ID NO: 84 - DNA, 15 bp, synthetic construct
  misc_feature 1..15: note = Synthetic polynucleotide
  misc_feature 1: note = LNA
  misc_feature 3..4: note = LNA
  misc_feature 6: note = LNA
  misc_feature 8..9: note = LNA
  misc_feature 12: note = LNA
  misc_feature 15: note = LNA
  source 1..15: mol_type = other DNA
tctagcatacttact

SEQ ID NO: 85 - DNA, 15 bp, synthetic construct
  misc_feature 1..15: note = Synthetic polynucleotide
  misc_feature 1..4: note = LNA
  misc_feature 12..15: note = LNA
  source 1..15: mol_type = other DNA
tctagcatacttact

SEQ ID NO: 86 - DNA, 15 bp, synthetic construct
  misc_feature 1..15: note = Synthetic polynucleotide
  misc_feature 1..3: note = LNA
  misc_feature 12..15: note = LNA
  source 1..15: mol_type = other DNA
gaattcggatggcca

SEQ ID NO: 87 - DNA, 15 bp, synthetic construct
  misc_feature 1..15: note = Synthetic polynucleotide
  misc_feature 1..4: note = LNA
  misc_feature 13..15: note = LNA
  source 1..15: mol_type = other DNA
ggccatcaattagtg

SEQ ID NO: 88 - DNA, 15 bp, synthetic construct
  misc_feature 1..15: note = Synthetic polynucleotide
  misc_feature 1..4: note = LNA
  misc_feature 13..15: note = LNA
  source 1..15: mol_type = other DNA
ttcggatggccatca

SEQ ID NO: 89 - DNA, 13 bp, synthetic construct
  misc_feature 1..13: note = Synthetic polynucleotide
  misc_feature 1..4: note = LNA
  misc_feature 11..13: note = LNA
  source 1..13: mol_type = other DNA
agccagacagcga

SEQ ID NO: 90 - DNA, 15 bp, synthetic construct
  misc_feature 1..15: note = Synthetic polynucleotide
  misc_feature 1..4: note = LNA
  misc_feature 13..15: note = LNA
  source 1..15: mol_type = other DNA
gacagccagacagca

SEQ ID NO: 91 - DNA, 15 bp, synthetic construct
  misc_feature 1..15: note = Synthetic polynucleotide
  source 1..15: mol_type = other DNA
tacttactgacagtc

SEQ ID NO: 92 - DNA, 15 bp, synthetic construct
  misc_feature 1..15: note = Synthetic polynucleotide
  source 1..15: mol_type = other DNA
tacttaccgacagcc

SEQ ID NO: 93 - DNA, 16 bp, synthetic construct
  misc_feature 1..16: note = Synthetic polynucleotide
  source 1..16: mol_type = other DNA
ggatttcggatggcca

SEQ ID NO: 94 - DNA, 15 bp, synthetic construct
  misc_feature 1..15: note = Synthetic polynucleotide
  misc_feature 1..4: note = LNA
  misc_feature 13..15: note = LNA
  source 1..15: mol_type = other DNA
tacttactgacagtc

SEQ ID NO: 95 - DNA, 15 bp, synthetic construct
  misc_feature 1..15: note = Synthetic polynucleotide
  misc_feature 1..4: note = LNA
  misc_feature 13..15: note = LNA
  source 1..15: mol_type = other DNA
tacttaccgacagcc

SEQ ID NO: 96 - DNA, 16 bp, synthetic construct
  misc_feature 1..16: note = Synthetic polynucleotide
  misc_feature 1..4: note = LNA
  misc_feature 14..16: note = LNA
  source 1..16: mol_type = other DNA
ggatttcggatggcca

SEQ ID NO: 97 - DNA, 26 bp, synthetic construct
  misc_feature 1..26: note = Synthetic polynucleotide
  source 1..26: mol_type = other DNA
agggctcttcggccagcraaagcagg

SEQ ID NO: 98 - DNA, 14 bp, synthetic construct
  misc_feature 1..14: note = synthetic sequence
  source 1..14: mol_type = other DNA
cgaccaaaagaatt

SEQ ID NO: 99 - DNA, 16 bp, synthetic construct
  misc_feature 1..16: note = synthetic sequence
  source 1..16: mol_type = other DNA
gaccaaaagaattcgg

SEQ ID NO: 100 - DNA, 16 bp, synthetic construct
  misc_feature 1..16: note = synthetic sequence
  source 1..16: mol_type = other DNA
agcatacttactgaca

SEQ ID NO: 101 - DNA, 14 bp, synthetic construct
  misc_feature 1..14: note = synthetic sequence
  source 1..14: mol_type = other DNA
catacttactgaca

SEQ ID NO: 102 - DNA, 14 bp, synthetic construct
  misc_feature 1..14: note = synthetic sequence
  source 1..14: mol_type = other DNA
atacttactgacag

SEQ ID NO: 103 - DNA, 16 bp, synthetic construct
  misc_feature 1..16: note = synthetic sequence
  source 1..16: mol_type = other DNA
catacttactgacagc

SEQ ID NO: 104 - DNA, 16 bp, synthetic construct
  misc_feature 1..16: note = synthetic sequence
  source 1..16: mol_type = other DNA
agacagcgaccaaaag

SEQ ID NO: 105 - DNA, 14 bp, synthetic construct
  misc_feature 1..14: note = synthetic sequence
  source 1..14: mol_type = other DNA
acagcgaccaaaag

SEQ ID NO: 106 - DNA, 15 bp, synthetic construct
  misc_feature 1..15: note = synthetic sequence
  source 1..15: mol_type = other DNA
cagccagacagcgac

SEQ ID NO: 107 - DNA, 14 bp, synthetic construct
  misc_feature 1..14: note = synthetic sequence
  source 1..14: mol_type = other DNA
cagccagacagcga

SEQ ID NO: 108 - DNA, 15 bp, synthetic construct
  misc_feature 1..15: note = synthetic sequence
  source 1..15: mol_type = other DNA
acagccagacagcga

SEQ ID NO: 109 - DNA, 15 bp, synthetic construct
  misc_feature 1..15: note = synthetic sequence
  source 1..15: mol_type = other DNA
gacagccagacagcg

SEQ ID NO: 110 - DNA, 15 bp, synthetic construct
  misc_feature 1..15: note = synthetic sequence
  source 1..15: mol_type = other DNA
catcaattagtgtcg

SEQ ID NO: 111 - DNA, 16 bp, synthetic construct
  misc_feature 1..16: note = synthetic sequence
  source 1..16: mol_type = other DNA
ccatcaattagtgtcg

SEQ ID NO: 112 - DNA, 16 bp, synthetic construct
  misc_feature 1..16: note = synthetic sequence
  source 1..16: mol_type = other DNA
gccatcaattagtgtg

SEQ ID NO: 113 - DNA, 15 bp, synthetic construct
  misc_feature 1..15: note = synthetic sequence
  source 1..15: mol_type = other DNA
aagaattcggatggc

SEQ ID NO: 114 - DNA, 14 bp, synthetic construct
  misc_feature 1..14: note = synthetic sequence
  source 1..14: mol_type = other DNA
cagacagcgaccaa

SEQ ID NO: 115 - DNA, 15 bp, synthetic construct
  misc_feature 1..15: note = synthetic sequence
  source 1..15: mol_type = other DNA
tgacagccagacagc

SEQ ID NO: 116 - DNA, 15 bp, synthetic construct
  misc_feature 1..15: note = synthetic sequence
  misc_feature 1..4: note = LNA
  misc_feature 12..15: note = LNA
  source 1..15: mol_type = other DNA
cagccagacagcgac

SEQ ID NO: 117 - DNA, 15 bp, synthetic construct
  misc_feature 1..15: note = synthetic sequence
  misc_feature 1..3: note = LNA
  misc_feature 12..15: note = LNA
  source 1..15: mol_type = other DNA
cagccagacagcgac

SEQ ID NO: 118 - DNA, 14 bp, synthetic construct
  misc_feature 1..14: note = synthetic sequence
  misc_feature 1..3: note = LNA
  misc_feature 11..14: note = LNA
  source 1..14: mol_type = other DNA
cagccagacagcga

SEQ ID NO: 119 - DNA, 14 bp, synthetic construct
  misc_feature 1..14: note = synthetic sequence
  misc_feature 1..3: note = LNA
  misc_feature 12..14: note = LNA
  source 1..14: mol_type = other DNA
cagccagacagcga

SEQ ID NO: 120 - DNA, 14 bp, synthetic construct
  misc_feature 1..14: note = synthetic sequence
  misc_feature 1..4: note = LNA
  misc_feature 12..14: note = LNA
  source 1..14: mol_type = other DNA
cagccagacagcga

SEQ ID NO: 121 - DNA, 15 bp, synthetic construct
  misc_feature 1..15: note = synthetic sequence
  misc_feature 1..3: note = LNA
  misc_feature 13..15: note = LNA
  source 1..15: mol_type = other DNA
acagccagacagcga

SEQ ID NO: 122 - DNA, 15 bp, synthetic construct
  misc_feature 1..15: note = synthetic sequence
  misc_feature 1..4: note = LNA
  misc_feature 12..15: note = LNA
  source 1..15: mol_type = other DNA
acagccagacagcga

SEQ ID NO: 123 - DNA, 15 bp, synthetic construct
  misc_feature 1..15: note = synthetic sequence
  misc_feature 1..3: note = LNA
  misc_feature 12..15: note = LNA
  source 1..15: mol_type = other DNA
acagccagacagcga

SEQ ID NO: 124 - DNA, 15 bp, synthetic construct
  misc_feature 1..15: note = synthetic sequence
  misc_feature 1..4: note = LNA
  misc_feature 13..15: note = LNA
  source 1..15: mol_type = other DNA
gacagccagacagcg

SEQ ID NO: 125 - DNA, 15 bp, synthetic construct
  misc_feature 1..15: note = synthetic sequence
  misc_feature 1..3: note = LNA
  misc_feature 13..15: note = LNA
  source 1..15: mol_type = other DNA
gacagccagacagcg

SEQ ID NO: 126 - DNA, 15 bp, synthetic construct
  misc_feature 1..15: note = synthetic sequence
  misc_feature 1..4: note = LNA
  misc_feature 12..15: note = LNA
  source 1..15: mol_type = other DNA
gacagccagacagcg

SEQ ID NO: 127 - DNA, 15 bp, synthetic construct
  misc_feature 1..15: note = synthetic sequence
  misc_feature 1..3: note = LNA
  misc_feature 13..15: note = LNA
  source 1..15: mol_type = other DNA
catcaattagtgtcg

SEQ ID NO: 128 - DNA, 16 bp, synthetic construct
  misc_feature 1..16: note = synthetic sequence
  misc_feature 1..3: note = LNA
  misc_feature 14..16: note = LNA
  source 1..16: mol_type = other DNA
ccatcaattagtgtcg

SEQ ID NO: 129 - DNA, 16 bp, synthetic construct
  misc_feature 1..16: note = synthetic sequence
  misc_feature 1..3: note = LNA
  misc_feature 14..16: note = LNA
  source 1..16: mol_type = other DNA
gccatcaattagtgtg

SEQ ID NO: 130 - DNA, 15 bp, synthetic construct
  misc_feature 1..15: note = synthetic sequence
  misc_feature 1..4: note = LNA
  misc_feature 12..15: note = LNA
  source 1..15: mol_type = other DNA
aagaattcggatggc

SEQ ID NO: 131 - DNA, 14 bp, synthetic construct
  misc_feature 1..14: note = synthetic sequence
  misc_feature 1..3: note = LNA
  misc_feature 12..14: note = LNA
  source 1..14: mol_type = other DNA
cagacagcgaccaa

SEQ ID NO: 132 - DNA, 15 bp, synthetic construct
  misc_feature 1..15: note = synthetic sequence
  misc_feature 1..3: note = LNA
  misc_feature 13..15: note = LNA
  source 1..15: mol_type = other DNA
tgacagccagacagc

SEQ ID NO: 133 - DNA, 15 bp, synthetic construct
  misc_feature 1..15: note = synthetic sequence
  misc_feature 1..4: note = LNA
  misc_feature 13..15: note = LNA
  source 1..15: mol_type = other DNA
gcgaccaaaagaatt

SEQ ID NO: 134 - DNA, 15 bp, synthetic construct
  misc_feature 1..15: note = synthetic sequence
  misc_feature 1..4: note = LNA
  misc_feature 12..15: note = LNA
  source 1..15: mol_type = other DNA
gcgaccaaaagaatt

SEQ ID NO: 135 - DNA, 14 bp, synthetic construct
  misc_feature 1..14: note = synthetic sequence
  misc_feature 1..4: note = LNA
  misc_feature 12..14: note = LNA
  source 1..14: mol_type = other DNA
cgaccaaaagaatt

SEQ ID NO: 136 - DNA, 15 bp, synthetic construct
  misc_feature 1..15: note = synthetic sequence
  misc_feature 1..3: note = LNA
  misc_feature 12..15: note = LNA
  source 1..15: mol_type = other DNA
cgaccaaaagaattc

SEQ ID NO: 137 - DNA, 15 bp, synthetic construct
  misc_feature 1..15: note = synthetic sequence
  misc_feature 1..4: note = LNA
  misc_feature 13..15: note = LNA
  source 1..15: mol_type = other DNA
cgaccaaaagaattc

SEQ ID NO: 138 - DNA, 15 bp, synthetic construct
  misc_feature 1..15: note = synthetic sequence
  misc_feature 1..3: note = LNA
  misc_feature 13..15: note = LNA
  source 1..15: mol_type = other DNA
cgaccaaaagaattc

SEQ ID NO: 139 - DNA, 14 bp, synthetic construct
  misc_feature 1..14: note = synthetic sequence
  misc_feature 1..3: note = LNA
  misc_feature 12..14: note = LNA
  source 1..14: mol_type = other DNA
gaccaaaagaattc

SEQ ID NO: 140 - DNA, 16 bp, synthetic construct
  misc_feature 1..16: note = synthetic sequence
  misc_feature 1..4: note = LNA
  misc_feature 13..16: note = LNA
  source 1..16: mol_type = other DNA
gcgaccaaaagaattc

SEQ ID NO: 141 - DNA, 16 bp, synthetic construct
  misc_feature 1..16: note = synthetic sequence
  misc_feature 1..3: note = LNA
  misc_feature 13..16: note = LNA
  source 1..16: mol_type = other DNA
gcgaccaaaagaattc

SEQ ID NO: 142 - DNA, 16 bp, synthetic construct
  misc_feature 1..16: note = synthetic sequence
  misc_feature 1..3: note = LNA
  misc_feature 14..16: note = LNA
  source 1..16: mol_type = other DNA
gcgaccaaaagaattc

SEQ ID NO: 143 - DNA, 16 bp, synthetic construct
  misc_feature 1..16: note = synthetic sequence
  misc_feature 1..3: note = LNA
  misc_feature 13..16: note = LNA
  source 1..16: mol_type = other DNA
cgaccaaaagaattcg

SEQ ID NO: 144 - DNA, 16 bp, synthetic construct
  misc_feature 1..16: note = synthetic sequence
  misc_feature 1..4: note = LNA
  misc_feature 13..16: note = LNA
  source 1..16: mol_type = other DNA
cgaccaaaagaattcg

SEQ ID NO: 145 - DNA, 14 bp, synthetic construct
  misc_feature 1..14: note = synthetic sequence
  misc_feature 1..3: note = LNA
  misc_feature 12..14: note = LNA
  source 1..14: mol_type = other DNA
gaccaaaagaattc

SEQ ID NO: 146 - DNA, 13 bp, synthetic construct
  misc_feature 1..13: note = synthetic sequence
  misc_feature 1..4: note = LNA
  misc_feature 11..13: note = LNA
  source 1..13: mol_type = other DNA
accaaaagaattc

SEQ ID NO: 147 - DNA, 17 bp, synthetic construct
  misc_feature 1..17: note = synthetic sequence
  misc_feature 1..3: note = LNA
  misc_feature 14..17: note = LNA
  source 1..17: mol_type = other DNA
cgaccaaaagaattcgg

SEQ ID NO: 148 - DNA, 16 bp, synthetic construct
  misc_feature 1..16: note = synthetic sequence
  misc_feature 1..3: note = LNA
  misc_feature 13..16: note = LNA
  source 1..16: mol_type = other DNA
gaccaaaagaattcgg

SEQ ID NO: 149 - DNA, 16 bp, synthetic construct
  misc_feature 1..16: note = synthetic sequence
  misc_feature 1..4: note = LNA
  misc_feature 14..16: note = LNA
  source 1..16: mol_type = other DNA
gaccaaaagaattcgg

SEQ ID NO: 150 - DNA, 16 bp, synthetic construct
  misc_feature 1..16: note = synthetic sequence
  misc_feature 1..3: note = LNA
  misc_feature 14..16: note = LNA
  source 1..16: mol_type = other DNA
gaccaaaagaattcgg

SEQ ID NO: 151 - DNA, 16 bp, synthetic construct
  misc_feature 1..16: note = synthetic sequence
  misc_feature 1..4: note = LNA
  misc_feature 13..16: note = LNA
  source 1..16: mol_type = other DNA
accaaaagaattcgga

SEQ ID NO: 152 - DNA, 15 bp, synthetic construct
  misc_feature 1..15: note = synthetic sequence
  misc_feature 1..4: note = LNA
  misc_feature 12..15: note = LNA
  source 1..15: mol_type = other DNA
ccaaaagaattcgga

SEQ ID NO: 153 - DNA, 14 bp, synthetic construct
  misc_feature 1..14: note = synthetic sequence
  misc_feature 1..4: note = LNA
  misc_feature 12..14: note = LNA
  source 1..14: mol_type = other DNA
caaaagaattcgga

SEQ ID NO: 154 - DNA, 14 bp, synthetic construct
  misc_feature 1..14: note = synthetic sequence
  misc_feature 1..3: note = LNA
  misc_feature 12..14: note = LNA
  source 1..14: mol_type = other DNA
caaaagaattcgga

SEQ ID NO: 155 - DNA, 16 bp, synthetic construct
  misc_feature 1..16: note = synthetic sequence
  misc_feature 1..3: note = LNA
  misc_feature 14..16: note = LNA
  source 1..16: mol_type = other DNA
ccaaaagaattcggat

SEQ ID NO: 156 - DNA, 16 bp, synthetic construct
  misc_feature 1..16: note = synthetic sequence
  misc_feature 1..4: note = LNA
  misc_feature 14..16: note = LNA
  source 1..16: mol_type = other DNA
ccaaaagaattcggat

SEQ ID NO: 157 - DNA, 15 bp, synthetic construct
  misc_feature 1..15: note = synthetic sequence
  misc_feature 1..4: note = LNA
  misc_feature 12..15: note = LNA
  source 1..15: mol_type = other DNA
caaaagaattcggat

SEQ ID NO: 158 - DNA, 15 bp, synthetic construct
  misc_feature 1..15: note = synthetic sequence
  misc_feature 1..3: note = LNA
  misc_feature 12..15: note = LNA
  source 1..15: mol_type = other DNA
caaaagaattcggat

SEQ ID NO: 159 - DNA, 16 bp, synthetic construct
  misc_feature 1..16: note = synthetic sequence
  misc_feature 1..4: note = LNA
  misc_feature 13..16: note = LNA
  source 1..16: mol_type = other DNA
agcatacttactgaca

SEQ ID NO: 160 - DNA, 14 bp, synthetic construct
  misc_feature 1..14: note = synthetic sequence
  misc_feature 1..3: note = LNA
  misc_feature 12..14: note = LNA
  source 1..14: mol_type = other DNA
catacttactgaca

SEQ ID NO: 161 - DNA, 15 bp, synthetic construct
  misc_feature 1..15: note = synthetic sequence
  misc_feature 1..4: note = LNA
  misc_feature 12..15: note = LNA
  source 1..15: mol_type = other DNA
catacttactgacag

SEQ ID NO: 162 - DNA, 14 bp, synthetic construct
  misc_feature 1..14: note = synthetic sequence
  misc_feature 1..3: note = LNA
  misc_feature 12..14: note = LNA
  source 1..14: mol_type = other DNA
atacttactgacag

SEQ ID NO: 163 - DNA, 14 bp, synthetic construct
  misc_feature 1..14: note = synthetic sequence
  misc_feature 1..4: note = LNA
  misc_feature 11..14: note = LNA
  source 1..14: mol_type = other DNA
atacttactgacag

SEQ ID NO: 164 - DNA, 14 bp, synthetic construct
  misc_feature 1..14: note = synthetic sequence
  misc_feature 1..3: note = LNA
  misc_feature 11..14: note = LNA
  source 1..14: mol_type = other DNA
atacttactgacag

SEQ ID NO: 165 - DNA, 16 bp, synthetic construct
  misc_feature 1..16: note = synthetic sequence
  misc_feature 1..4: note = LNA
  misc_feature 13..16: note = LNA
  source 1..16: mol_type = other DNA
catacttactgacagc

SEQ ID NO: 166 - DNA, 16 bp, synthetic construct
  misc_feature 1..16: note = synthetic sequence
  misc_feature 1..3: note = LNA
  misc_feature 13..16: note = LNA
  source 1..16: mol_type = other DNA
catacttactgacagc

SEQ ID NO: 167 - DNA, 16 bp, synthetic construct
  misc_feature 1..16: note = synthetic sequence
  misc_feature 1..4: note = LNA
  misc_feature 14..16: note = LNA
  source 1..16: mol_type = other DNA
catacttactgacagc

SEQ ID NO: 168 - DNA, 15 bp, synthetic construct
  misc_feature 1..15: note = synthetic sequence
  misc_feature 1..3: note = LNA
  misc_feature 13..15: note = LNA
  source 1..15: mol_type = other DNA
atacttactgacagc

SEQ ID NO: 169 - DNA, 15 bp, synthetic construct
  misc_feature 1..15: note = synthetic sequence
  misc_feature 1..4: note = LNA
  misc_feature 12..15: note = LNA
  source 1..15: mol_type = other DNA
atacttactgacagc

SEQ ID NO: 170 - DNA, 15 bp, synthetic construct
  misc_feature 1..15: note = synthetic sequence
  misc_feature 1..4: note = LNA
  misc_feature 13..15: note = LNA
  source 1..15: mol_type = other DNA
atacttactgacagc

SEQ ID NO: 171 - DNA, 15 bp, synthetic construct
  misc_feature 1..15: note = synthetic sequence
  misc_feature 1..3: note = LNA
  misc_feature 12..15: note = LNA
  source 1..15: mol_type = other DNA
atacttactgacagc

SEQ ID NO: 172 - DNA, 14 bp, synthetic construct
  misc_feature 1..14: note = synthetic sequence
  misc_feature 1..3: note = LNA
  misc_feature 12..14: note = LNA
  source 1..14: mol_type = other DNA
tacttactgacagc

SEQ ID NO: 173 - DNA, 14 bp, synthetic construct
  misc_feature 1..14: note = synthetic sequence
  misc_feature 1..3: note = LNA
  misc_feature 11..14: note = LNA
  source 1..14: mol_type = other DNA
tacttactgacagc

SEQ ID NO: 174 - DNA, 14 bp, synthetic construct
  misc_feature 1..14: note = synthetic sequence
  misc_feature 1..4: note = LNA
  misc_feature 11..14: note = LNA
  source 1..14: mol_type = other DNA
tacttactgacagc

SEQ ID NO: 175 - DNA, 16 bp, synthetic construct
  misc_feature 1..16: note = synthetic sequence
  misc_feature 1..3: note = LNA
  misc_feature 14..16: note = LNA
  source 1..16: mol_type = other DNA
atacttactgacagcc

SEQ ID NO: 176 - DNA, 16 bp, synthetic construct
  misc_feature 1..16: note = synthetic sequence
  misc_feature 1..3: note = LNA
  misc_feature 13..16: note = LNA
  source 1..16: mol_type = other DNA
atacttactgacagcc

SEQ ID NO: 177 - DNA, 15 bp, synthetic construct
  misc_feature 1..15: note = synthetic sequence
  misc_feature 1..4: note = LNA
  misc_feature 12..15: note = LNA
  source 1..15: mol_type = other DNA
tacttactgacagcc

SEQ ID NO: 178 - DNA, 15 bp, synthetic construct
  misc_feature 1..15: note = synthetic sequence
  misc_feature 1..3: note = LNA
  misc_feature 13..15: note = LNA
  source 1..15: mol_type = other DNA
tacttactgacagcc

SEQ ID NO: 179 - DNA, 16 bp, synthetic construct
  misc_feature 1..16: note = synthetic sequence
  misc_feature 1..4: note = LNA
  misc_feature 13..16: note = LNA
  source 1..16: mol_type = other DNA
tacttactgacagcca

SEQ ID NO: 180 - DNA, 16 bp, synthetic construct
  misc_feature 1..16: note = synthetic sequence
  misc_feature 1..3: note = LNA
  misc_feature 13..16: note = LNA
  source 1..16: mol_type = other DNA
tacttactgacagcca

SEQ ID NO: 181 - DNA, 16 bp, synthetic construct
  misc_feature 1..16: note = synthetic sequence
  misc_feature 1..4: note = LNA
  misc_feature 14..16: note = LNA
  source 1..16: mol_type = other DNA
tacttactgacagcca

SEQ ID NO: 182 - DNA, 16 bp, synthetic construct
  misc_feature 1..16: note = synthetic sequence
  misc_feature 1..3: note = LNA
  misc_feature 14..16: note = LNA
  source 1..16: mol_type = other DNA
tacttactgacagcca

SEQ ID NO: 183 - DNA, 15 bp, synthetic construct
  misc_feature 1..15: note = synthetic sequence
  misc_feature 1..3: note = LNA
  misc_feature 12..15: note = LNA
  source 1..15: mol_type = other DNA
acttactgacagcca

SEQ ID NO: 184 - DNA, 15 bp, synthetic construct
  misc_feature 1..15: note = synthetic sequence
  misc_feature 1..3: note = LNA
  misc_feature 13..15: note = LNA
  source 1..15: mol_type = other DNA
acttactgacagcca

SEQ ID NO: 185 - DNA, 15 bp, synthetic construct
  misc_feature 1..15: note = synthetic sequence
  misc_feature 1..4: note = LNA
  misc_feature 12..15: note = LNA
  source 1..15: mol_type = other DNA
acttactgacagcca

SEQ ID NO: 186 - DNA, 15 bp, synthetic construct
  misc_feature 1..15: note = synthetic sequence
  misc_feature 1..4: note = LNA
  misc_feature 12..15: note = LNA
  source 1..15: mol_type = other DNA
cttactgacagccag

SEQ ID NO: 187 - DNA, 15 bp, synthetic construct
  misc_feature 1..15: note = synthetic sequence
  misc_feature 1..3: note = LNA
  misc_feature 13..15: note = LNA
  source 1..15: mol_type = other DNA
ttactgacagccaga

SEQ ID NO: 188 - DNA, 16 bp, synthetic construct
  misc_feature 1..16: note = synthetic sequence
  misc_feature 1..3: note = LNA
  misc_feature 14..16: note = LNA
  source 1..16: mol_type = other DNA
agacagcgaccaaaag

SEQ ID NO: 189 - DNA, 16 bp, synthetic construct
  misc_feature 1..16: note = synthetic sequence
  misc_feature 1..4: note = LNA
  misc_feature 13..16: note = LNA
  source 1..16: mol_type = other DNA
agacagcgaccaaaag

SEQ ID NO: 190 - DNA, 14 bp, synthetic construct
  misc_feature 1..14: note = synthetic sequence
  misc_feature 1..4: note = LNA
  misc_feature 11..14: note = LNA
  source 1..14: mol_type = other DNA
acagcgaccaaaag

SEQ ID NO: 191 - DNA, 14 bp, synthetic construct
  misc_feature 1..14: note = synthetic sequence
  misc_feature 1..3: note = LNA
  misc_feature 12..14: note = LNA
  source 1..14: mol_type = other DNA
acagcgaccaaaag

SEQ ID NO: 192 - DNA, 28 bp, SARS-CoV-2
  source 1..28: mol_type = other DNA
ggtgacatggtaccacatatatcacgtc

SEQ ID NO: 193 - DNA, 28 bp, SARS-CoV-2
  source 1..28: mol_type = other DNA
gacgtgatatatgtggtaccatgtcacc

SEQ ID NO: 194 - DNA, 16 bp, SARS-CoV-2
  source 1..16: mol_type = other DNA
gacgtgatatatgtgg

SEQ ID NO: 195 - DNA, 16 bp, SARS-CoV-2
  source 1..16: mol_type = other DNA
cgtgatatatgtggta

SEQ ID NO: 196 - DNA, 15 bp, SARS-CoV-2
  source 1..15: mol_type = other DNA
gatatgtggtaccat

SEQ ID NO: 197 - DNA, 14 bp, SARS-CoV-2
  source 1..14: mol_type = other DNA
tggtaccatgtcac

SEQ ID NO: 198 - DNA, 25 bp, SARS-CoV-2
  source 1..25: mol_type = other DNA
gtcactaagaaatctgctgctgagg

SEQ ID NO: 199 - DNA, 25 bp, SARS-CoV-2
  source 1..25: mol_type = other DNA
cctcagcagcagatttcttagtgac

SEQ ID NO: 200 - DNA, 16 bp, SARS-CoV-2
  source 1..16: mol_type = other DNA
cctcagcagcagattt

SEQ ID NO: 201 - DNA, 15 bp, SARS-CoV-2
  source 1..15: mol_type = other DNA
tcagcagcagatttc

SEQ ID NO: 202 - DNA, 14 bp, SARS-CoV-2
  source 1..14: mol_type = other DNA
cagcagcagatttc

SEQ ID NO: 203 - DNA, 16 bp, SARS-CoV-2
  source 1..16: mol_type = other DNA
cagatttcttagtgac

SEQ ID NO: 204 - DNA, 25 bp, SARS-CoV-2
  source 1..25: mol_type = other DNA
tgcttacggtttcgtccgtgttgca

SEQ ID NO: 205 - DNA, 25 bp, SARS-CoV-2
  source 1..25: mol_type = other DNA
tgcaacacggacgaaaccgtaagca

SEQ ID NO: 206 - DNA, 16 bp, SARS-CoV-2
  source 1..16: mol_type = other DNA
tgcaacacggacgaaa

SEQ ID NO: 207 - DNA, 16 bp, SARS-CoV-2
  source 1..16: mol_type = other DNA
gcaacacggacgaaac

SEQ ID NO: 208 - DNA, 15 bp, SARS-CoV-2
  source 1..15: mol_type = other DNA
acacggacgaaaccg

SEQ ID NO: 209 - DNA, 15 bp, SARS-CoV-2
  source 1..15: mol_type = other DNA
ggacgaaacccgtaa

SEQ ID NO: 210 - DNA, 15 bp, SARS-CoV-2
  source 1..15: mol_type = other DNA
acgaaaccgtaagca

SEQ ID NO: 211 - DNA, 15 bp, SARS-CoV-2
  source 1..15: mol_type = other DNA
acgaaaccgtaagca

SEQ ID NO: 212 - DNA, 16 bp, SARS-CoV-2
  source 1..16: mol_type = other DNA
gcaacacggacgaaac

SEQ ID NO: 213 - DNA, 15 bp, SARS-CoV-2
  source 1..15: mol_type = other DNA
gcaacacggacgaaa

SEQ ID NO: 214 - DNA, 16 bp, SARS-CoV-2
  source 1..16: mol_type = other DNA
gcaacacggacgaaac

SEQ ID NO: 215 - DNA, 16 bp, SARS-CoV-2
  source 1..16: mol_type = other DNA
gcaacacggacgaaac

SEQ ID NO: 216 - DNA, 16 bp, SARS-CoV-2
  source 1..16: mol_type = other DNA
gcaacacggacgaaac

SEQ ID NO: 217 - DNA, 14 bp, SARS-CoV-2
  source 1..14: mol_type = other DNA
gcaacacggacgaa

SEQ ID NO: 218 - DNA, 15 bp, SARS-CoV-2
  source 1..15: mol_type = other DNA
acacggacgaaaccg

SEQ ID NO: 219 - DNA, 15 bp, SARS-CoV-2
  source 1..15: mol_type = other DNA
acacggacgaaaccg

SEQ ID NO: 220 - DNA, 16 bp, SARS-CoV-2
  source 1..16: mol_type = other DNA
aacacggacgaaaccg

SEQ ID NO: 221 - DNA, 16 bp, SARS-CoV-2
  source 1..16: mol_type = other DNA
aacacggacgaaaccg

SEQ ID NO: 222 - DNA, 15 bp, SARS-CoV-2
  source 1..15: mol_type = other DNA
acgaaaccgtaagca

SEQ ID NO: 223 - DNA, 15 bp, SARS-CoV-2
  source 1..15: mol_type = other DNA
acgaaaccgtaagca

SEQ ID NO: 224 - DNA, 19 bp, SARS-CoV-2
  source 1..19: mol_type = other DNA
ataggtccagacatgttcc

SEQ ID NO: 225 - DNA, 19 bp, SARS-CoV-2
  source 1..19: mol_type = other DNA
ggaacatgtctggacctat

SEQ ID NO: 226 - DNA, 16 bp, SARS-CoV-2
  source 1..16: mol_type = other DNA
aacatgtctggaccta

SEQ ID NO: 227 - DNA, 16 bp, SARS-CoV-2
  source 1..16: mol_type = other DNA
acatgtctggacctat

SEQ ID NO: 228 - DNA, 19 bp, SARS-CoV-2
  source 1..19: mol_type = other DNA
tatgactatgtcatattca

SEQ ID NO: 229 - DNA, 23 bp, SARS-CoV-2
  source 1..23: mol_type = other DNA
agtgaatatgacatagtcatatt

SEQ ID NO: 230 - DNA, 15 bp, SARS-CoV-2
  source 1..15: mol_type = other DNA
tgaatatgacatagt

SEQ ID NO: 231 - DNA, 14 bp, SARS-CoV-2
  source 1..14: mol_type = other DNA
aatatgacatagtc

SEQ ID NO: 232 - DNA, 44 bp, SARS-CoV-2
  source 1..44: mol_type = other DNA
gatctcttgtagatctgttctctaaacgaactttaaaatctgtg

SEQ ID NO: 233 - DNA, 44 bp, SARS-CoV-2
  source 1..44: mol_type = other DNA
cacagattttaaagttcgtttagagaacagatctacaagagatc

SEQ ID NO: 234 - DNA, 16 bp, SARS-CoV-2
  source 1..16: mol_type = other DNA
cacagattttaaagtt

SEQ ID NO: 235 - DNA, 16 bp, SARS-CoV-2
  source 1..16: mol_type = other DNA
cacagattttaaagtt

SEQ ID NO: 236 - DNA, 16 bp, SARS-CoV-2
  source 1..16: mol_type = other DNA
cagattttaaagttcg

SEQ ID NO: 237 - DNA, 15 bp, SARS-CoV-2
  source 1..15: mol_type = other DNA
gattttaaagttcgt

SEQ ID NO: 238 - DNA, 15 bp, SARS-CoV-2
  source 1..15: mol_type = other DNA
taaagttcgtttaga

SEQ ID NO: 239 - DNA, 14 bp, SARS-CoV-2
  source 1..14: mol_type = other DNA
aaagttcgtttaga

SEQ ID NO: 240 - DNA, 17 bp, SARS-CoV-2
  source 1..17: mol_type = other DNA
tcgtttagagaacagat

SEQ ID NO: 241 - DNA, 16 bp, SARS-CoV-2
  source 1..16: mol_type = other DNA
agagaacagatctaca

SEQ ID NO: 242 - DNA, 14 bp, SARS-CoV-2
  source 1..14: mol_type = other DNA
agatctacaagaga

SEQ ID NO: 243 - DNA, 14 bp, SARS-CoV-2
  source 1..14: mol_type = other DNA
atctacaagagatc

SEQ ID NO: 244 - DNA, 16 bp, SARS-CoV-2
  source 1..16: mol_type = other DNA
agattttaaagttcgt

SEQ ID NO: 245 - DNA, 15 bp, SARS-CoV-2
  source 1..15: mol_type = other DNA
gattttaaagttcgt

SEQ ID NO: 246 - DNA, 15 bp, SARS-CoV-2
  source 1..15: mol_type = other DNA
gattttaaagttcgt

SEQ ID NO: 247 - DNA, 15 bp, SARS-CoV-2
  source 1..15: mol_type = other DNA
agattttaaagttcg

SEQ ID NO: 248 - DNA, 17 bp, SARS-CoV-2
  source 1..17: mol_type = other DNA
tcgtttagagaacagat

SEQ ID NO: 249 - DNA, 16 bp, SARS-CoV-2
  source 1..16: mol_type = other DNA
ttcgtttagagaacag

SEQ ID NO: 250 - DNA, 16 bp, SARS-CoV-2
  source 1..16: mol_type = other DNA
ttcgtttagagaacag

SEQ ID NO: 251 - DNA, 31 bp, SARS-CoV-2
  source 1..31: mol_type = other DNA
gagaaaacacacgtccaactcagtttgcctg

SEQ ID NO: 252 - DNA, 31 bp, SARS-CoV-2
  source 1..31: mol_type = other DNA
caggcaaactgagttggacgtgtgttttctc

SEQ ID NO: 253 - DNA, 16 bp, SARS-CoV-2
  source 1..16: mol_type = other DNA
caggcaaactgagttg

SEQ ID NO: 254 - DNA, 16 bp, SARS-CoV-2
  source 1..16: mol_type = other DNA
caggcaaactgagttg

SEQ ID NO: 255 - DNA, 14 bp, SARS-CoV-2
  source 1..14: mol_type = other DNA
caggcaaactgagt

SEQ ID NO: 256 - DNA, 16 bp, SARS-CoV-2
  source 1..16: mol_type = other DNA
caaactgagttggacg

SEQ ID NO: 257 - DNA, 14 bp, SARS-CoV-2
  source 1..14: mol_type = other DNA
aaactgagttggac

SEQ ID NO: 258 - DNA, 16 bp, SARS-CoV-2
  source 1..16: mol_type = other DNA
aaactgagttggacgt

SEQ ID NO: 259 - DNA, 15 bp, SARS-CoV-2
  source 1..15: mol_type = other DNA
gagttggacgtgtgt

SEQ ID NO: 260 - DNA, 16 bp, SARS-CoV-2
  source 1..16: mol_type = other DNA
ttggacgtgtgttttc

SEQ ID NO: 261 - DNA, 16 bp, SARS-CoV-2
  source 1..16: mol_type = other DNA
ggacgtgtgttttctc

SEQ ID NO: 262 - DNA, 21 bp, SARS-CoV-2
  source 1..21: mol_type = other DNA
ggtttcgtccgggtgtgaccg

SEQ ID NO: 263 - DNA, 29 bp, SARS-CoV-2
  source 1..29: mol_type = other DNA
tttcggtcacacccggacgaaacctagat

SEQ ID NO: 264 - DNA, 16 bp, SARS-CoV-2
  source 1..16: mol_type = other DNA
tttcggtcacacccgg

SEQ ID NO: 265 - DNA, 16 bp, SARS-CoV-2
  source 1..16: mol_type = other DNA
cggtcacacccggacg

SEQ ID NO: 266 - DNA, 16 bp, SARS-CoV-2
  source 1..16: mol_type = other DNA
tcacacccggacgaaa

SEQ ID NO: 267 - DNA, 14 bp, SARS-CoV-2
  source 1..14: mol_type = other DNA
cacccggacgaaac

SEQ ID NO: 268 - DNA, 15 bp, SARS-CoV-2
  source 1..15: mol_type = other DNA
cacccggacgaaacc

SEQ ID NO: 269 - DNA, 16 bp, SARS-CoV-2
  source 1..16: mol_type = other DNA
cacccggacgaaacct

SEQ ID NO: 270 - DNA, 14 bp, SARS-CoV-2
  source 1..14: mol_type = other DNA
ccggacgaaaccta

SEQ ID NO: 271 - DNA, 17 bp, SARS-CoV-2
  source 1..17: mol_type = other DNA
cggtcacacccggacga

SEQ ID NO: 272 - DNA, 16 bp, SARS-CoV-2
  source 1..16: mol_type = other DNA
cggtcacacccggacg

SEQ ID NO: 273 - DNA, 16 bp, SARS-CoV-2
  source 1..16: mol_type = other DNA
cggtcacacccggacg

SEQ ID NO: 274 - DNA, 16 bp, SARS-CoV-2
  source 1..16: mol_type = other DNA
cggtcacacccggacg

SEQ ID NO: 275 - DNA, 14 bp, SARS-CoV-2
  source 1..14: mol_type = other DNA
gtcacacccggacg

SEQ ID NO: 276 - DNA, 14 bp, SARS-CoV-2
  source 1..14: mol_type = other DNA
gtcacacccggacg

SEQ ID NO: 277 - DNA, 15 bp, SARS-CoV-2
  source 1..15: mol_type = other DNA
cacccggacgaaacc

SEQ ID NO: 278 - DNA, 15 bp, SARS-CoV-2
  source 1..15: mol_type = other DNA
cacccggacgaaacc

SEQ ID NO: 279 - DNA, 14 bp, SARS-CoV-2
  source 1..14: mol_type = other DNA
cacccggacgaaac

SEQ ID NO: 280 - DNA, 16 bp, SARS-CoV-2
  source 1..16: mol_type = other DNA
cacacccggacgaaac

SEQ ID NO: 281 - DNA, 15 bp, SARS-CoV-2
  source 1..15: mol_type = other DNA
cacacccggacgaaa

SEQ ID NO: 282 - DNA, 14 bp, SARS-CoV-2
  source 1..14: mol_type = other DNA
cacacccggacgaa

SEQ ID NO: 283 - DNA, 24 bp, SARS-CoV-2
  source 1..24: mol_type = other DNA
cgaggccacgcggagtacgatcga

SEQ ID NO: 284 - DNA, 31 bp, SARS-CoV-2
  source 1..31: mol_type = other DNA
actcgatcgtactccgcgtggcctcggtgaa

SEQ ID NO: 285 - DNA, 15 bp, SARS-CoV-2
  source 1..15: mol_type = other DNA
tcgatcgtactccgc

SEQ ID NO: 286 - DNA, 14 bp, SARS-CoV-2
  source 1..14: mol_type = other DNA
tcgatcgtactccg

SEQ ID NO: 287 - DNA, 15 bp, SARS-CoV-2
  source 1..15: mol_type = other DNA
atcgtactccgcgtg

SEQ ID NO: 288 - DNA, 14 bp, SARS-CoV-2
  source 1..14: mol_type = other DNA
actcgatcgtactc

SEQ ID NO: 289 - DNA, 15 bp, SARS-CoV-2
  source 1..15: mol_type = other DNA
cgtggcctcggtgaa

SEQ ID NO: 290 - DNA, 14 bp, SARS-CoV-2
  source 1..14: mol_type = other DNA
gtggcctcggtgaa

SEQ ID NO: 291 - DNA, 35 bp, SARS-CoV-2
  source 1..35: mol_type = other DNA
tagttaactttaatctcacatagcaatctttaatc

SEQ ID NO: 292 - DNA, 35 bp, SARS-CoV-2
  source 1..35: mol_type = other DNA
gattaaagattgctatgtgagattaaagttaacta

SEQ ID NO: 293 - DNA, 16 bp, SARS-CoV-2
  source 1..16: mol_type = other DNA
gattaaagattgctat

SEQ ID NO: 294 - DNA, 16 bp, SARS-CoV-2
  source 1..16: mol_type = other DNA
taaagattgctatgtg

SEQ ID NO: 295 - DNA, 16 bp, SARS-CoV-2
  source 1..16: mol_type = other DNA
aagattgctatgtgag

SEQ ID NO: 296 - DNA, 16 bp, SARS-CoV-2
  source 1..16: mol_type = other DNA
gctatgtgagttaaag

SEQ ID NO: 297 - DNA, 16 bp, SARS-CoV-2
  source 1..16: mol_type = other DNA
tatgtgagttaaagtt

SEQ ID NO: 298 - DNA, 16 bp, SARS-CoV-2
  source 1..16: mol_type = other DNA
tgtgagttaaagttaa

SEQ ID NO: 299 - DNA, 50 bp, SARS-CoV-2
  source 1..50: mol_type = other DNA
cgtgctacaacttcctcaaggaacaacattgccaaaaggcttctacgcag

SEQ ID NO: 300 - DNA, 50 bp, SARS-CoV-2
  source 1..50: mol_type = other DNA
ctgcgtagaagccttttggcaatgttgttccttgaggaagttgtagcacg

SEQ ID NO: 301 - DNA, 16 bp, SARS-CoV-2
  source 1..16: mol_type = other DNA
tcgtagaagccttttg

SEQ ID NO: 302 - DNA, 17 bp, SARS-CoV-2
  source 1..17: mol_type = other DNA
cgtagaagccttttggc

SEQ ID NO: 303 - DNA, 16 bp, SARS-CoV-2
  source 1..16: mol_type = other DNA
tagaagccttttggca

SEQ ID NO: 304 - DNA, 16 bp, SARS-CoV-2
  source 1..16: mol_type = other DNA
aagccttttggcaatg

SEQ ID NO: 305 - DNA, 16 bp, SARS-CoV-2
  source 1..16: mol_type = other DNA
ttggcaatgttgttcc

SEQ ID NO: 306 - DNA, 14 bp, SARS-CoV-2
  source 1..14: mol_type = other DNA
gcaatgttgttcct

SEQ ID NO: 307 - DNA, 14 bp, SARS-CoV-2
  source 1..14: mol_type = other DNA
cttgaggaagttgt

SEQ ID NO: 308 - DNA, 16 bp, SARS-CoV-2
  source 1..16: mol_type = other DNA
aggaagttgtagcacg

SEQ ID NO: 309 - DNA, 43 bp, SARS-CoV-2
  source 1..43: mol_type = other DNA
gcctatatggaagagccctaatgtgtaaaattaattttagtag

SEQ ID NO: 310 - DNA, 43 bp, SARS-CoV-2
  source 1..43: mol_type = other DNA
ctactaaaattaattttacacattagggctcttccatataggc

SEQ ID NO: 311 - DNA, 15 bp, SARS-CoV-2
  source 1..15: mol_type = other DNA
ctactaaaattaatt

SEQ ID NO: 312 - DNA, 15 bp, SARS-CoV-2
  source 1..15: mol_type = other DNA
tactaaaattaattt

SEQ ID NO: 313 - DNA, 14 bp, SARS-CoV-2
  source 1..14: mol_type = other DNA
actaaaattaattt

SEQ ID NO: 314 - DNA, 16 bp, SARS-CoV-2
  source 1..16: mol_type = other DNA
aattaattttacacat

SEQ ID NO: 315 - DNA, 16 bp, SARS-CoV-2
  source 1..16: mol_type = other DNA
attttacacattaggg

SEQ ID NO: 316 - DNA, 15 bp, SARS-CoV-2
  source 1..15: mol_type = other DNA
tacacattagggctc

SEQ ID NO: 317 - DNA, 15 bp, SARS-CoV-2
  source 1..15: mol_type = other DNA
acattagggctcttc

SEQ ID NO: 318 - DNA, 15 bp, SARS-CoV-2
  source 1..15: mol_type = other DNA
tagggctcttccata

SEQ ID NO: 319 - DNA, 15 bp, SARS-CoV-2
  source 1..15: mol_type = other DNA
gctcttccatatagg

SEQ ID NO: 320 - DNA, 19 bp, SARS-CoV-2
  source 1..19: mol_type = other DNA
aggtaagatggagagcctt

SEQ ID NO: 321 - DNA, 24 bp, SARS-CoV-2
  source 1..24: mol_type = other DNA
aaggctctccatcttacctttcgg

SEQ ID NO: 322 - DNA, 16 bp, SARS-CoV-2
  source 1..16: mol_type = other DNA
aaggctctccatctta

SEQ ID NO: 323 - DNA, 14 bp, SARS-CoV-2
  source 1..14: mol_type = other DNA
aaggctctccatct

SEQ ID NO: 324 - DNA, 16 bp, SARS-CoV-2
  source 1..16: mol_type = other DNA
gctctccatcttacct

SEQ ID NO: 325 - DNA, 16 bp, SARS-CoV-2
  source 1..16: mol_type = other DNA
tccatcttacctttcg

SEQ ID NO: 326 - DNA, 18 bp, SARS-CoV-2
  source 1..18: mol_type = other DNA
tgtgtaacattagggagg

SEQ ID NO: 327 - DNA, 18 bp, SARS-CoV-2
  source 1..18: mol_type = other DNA
cctccctaatgttacaca

SEQ ID NO: 328 - DNA, 16 bp, SARS-CoV-2
  source 1..16: mol_type = other DNA
cctccctaatgttaca

SEQ ID NO: 329 - DNA, 16 bp, SARS-CoV-2
  source 1..16: mol_type = other DNA
ctccctaatgttacag

SEQ ID NO: 330 - DNA, 16 bp, SARS-CoV-2
  source 1..16: mol_type = other DNA
ctccctaatgttacag

SEQ ID NO: 331 - DNA, 22 bp, SARS-CoV-2
  source 1..22: mol_type = other DNA
tcatgtggtagtgttggtttta

SEQ ID NO: 332 - DNA, 22 bp, SARS-CoV-2
  source 1..22: mol_type = other DNA
taaaaccaacactaccacatga

SEQ ID NO: 333 - DNA, 16 bp, SARS-CoV-2
  source 1..16: mol_type = other DNA
taaaaccaacactacc

SEQ ID NO: 334 - DNA, 16 bp, SARS-CoV-2
  source 1..16: mol_type = other DNA
aaaccaacactaccac

SEQ ID NO: 335 - DNA, 16 bp, SARS-CoV-2
  source 1..16: mol_type = other DNA
aaaccaacactaccac

SEQ ID NO: 336 - DNA, 16 bp, SARS-CoV-2
  source 1..16: mol_type = other DNA
accaacactaccacat

SEQ ID NO: 337 - DNA, 14 bp, influenza A virus
  source 1..14: mol_type = other DNA
tgtcagtaagtatg

SEQ ID NO: 338 - DNA, 16 bp, influenza A virus
  source 1..16: mol_type = other DNA
ctggctgtcagtaagt

SEQ ID NO: 339 - DNA, 15 bp, influenza A virus
  source 1..15: mol_type = other DNA
tcgctgtctggctgt

SEQ ID NO: 340 - DNA, 16 bp, influenza A virus
  source 1..16: mol_type = other DNA
cttttggtcgctgtct

SEQ ID NO: 341 - DNA, 14 bp, influenza A virus
  source 1..14: mol_type = other DNA
cttttggtcgctgt

SEQ ID NO: 342 - DNA, 16 bp, influenza A virus
  source 1..16: mol_type = other DNA
ttggtcgctgtctggc

SEQ ID NO: 343 - DNA, 14 bp, influenza A virus
  source 1..14: mol_type = other DNA
ttggtcgctgtctg

SEQ ID NO: 344 - DNA, 16 bp, influenza A virus
  source 1..16: mol_type = other DNA
gaattcttttggtcgc

SEQ ID NO: 345 - DNA, 15 bp, influenza A virus
  source 1..15: mol_type = other DNA
gaattcttttggtcg

SEQ ID NO: 346 - DNA, 15 bp, influenza A virus
  source 1..15: mol_type = other DNA
aattcttttggtcgc

SEQ ID NO: 347 - DNA, 16 bp, influenza A virus
  source 1..16: mol_type = other DNA
cgaattcttttggtcg

SEQ ID NO: 348 - DNA, 15 bp, influenza A virus
  source 1..15: mol_type = other DNA
acactaattgatggc

SEQ ID NO: 349 - DNA, 13 bp, influenza A virus
  source 1..13: mol_type = other DNA
aattgatggccat

SEQ ID NO: 350 - DNA, 16 bp, influenza B virus
  source 1..16: mol_type = other DNA
ccacaaaatgaaggca

SEQ ID NO: 351 - DNA, 15 bp, influenza B virus
  source 1..15: mol_type = other DNA
cacaaaatgaaggca

SEQ ID NO: 352 - DNA, 14 bp, influenza B virus
  source 1..14: mol_type = other DNA
cacaaaatgaaggc

SEQ ID NO: 353 - DNA, 14 bp, influenza B virus
  source 1..14: mol_type = other DNA
caataattgtacta

SEQ ID NO: 354 - DNA, 14 bp, influenza B virus
  source 1..14: mol_type = other DNA
caataattgtacta

SEQ ID NO: 355 - DNA, 14 bp, influenza B virus
  source 1..14: mol_type = other DNA
caataattgtacta

SEQ ID NO: 356 - DNA, 15 bp, influenza B virus
  source 1..15: mol_type = other DNA
caataattgtactac

SEQ ID NO: 357 - DNA, 15 bp, influenza B virus
  source 1..15: mol_type = other DNA
caataattgtactac

SEQ ID NO: 358 - DNA, 16 bp, influenza B virus
  source 1..16: mol_type = other DNA
tgtactactcatggta

SEQ ID NO: 359 - DNA, 16 bp, influenza B virus
  source 1..16: mol_type = other DNA
tgtactactcatggta

SEQ ID NO: 360 - DNA, 16 bp, influenza B virus
  source 1..16: mol_type = other DNA
tgtactactcatggta

SEQ ID NO: 361 - DNA, 14 bp, influenza B virus
  source 1..14: mol_type = other DNA
gtactactcatggt

SEQ ID NO: 362 - DNA, 15 bp, influenza B virus
  source 1..15: mol_type = other DNA
ttgtactactcatgg

SEQ ID NO: 363 - DNA, 15 bp, influenza B virus
  source 1..15: mol_type = other DNA
catggtagtaacatc

SEQ ID NO: 364 - DNA, 17 bp, influenza B virus
  source 1..17: mol_type = other DNA
ctcatggtagtaacatc

SEQ ID NO: 365 - DNA, 16 bp, influenza B virus
  source 1..16: mol_type = other DNA
ctcatggtagtaacat

SEQ ID NO: 366 - DNA, 16 bp, influenza B virus
  source 1..16: mol_type = other DNA
ctcatggtagtaacat

SEQ ID NO: 367 - DNA, 16 bp, influenza B virus
  source 1..16: mol_type = other DNA
actcatggtagtaaca

SEQ ID NO: 368 - DNA, 16 bp, influenza B virus
  source 1..16: mol_type = other DNA
actcatggtagtaaca

SEQ ID NO: 369 - DNA, 15 bp, influenza B virus
  source 1..15: mol_type = other DNA
actcatggtagtaac

SEQ ID NO: 370 - DNA, 14 bp, influenza B virus
  source 1..14: mol_type = other DNA
actcatggtagtaa

SEQ ID NO: 371 - DNA, 15 bp, influenza B virus
  source 1..15: mol_type = other DNA
caatgcagatcgaat

SEQ ID NO: 372 - DNA, 15 bp, influenza B virus
  source 1..15: mol_type = other DNA
caatgcagatcgaat

SEQ ID NO: 373 - DNA, 16 bp, influenza B virus
  source 1..16: mol_type = other DNA
gattgccttcacgaaa

SEQ ID NO: 374 - DNA, 16 bp, influenza B virus
  source 1..16: mol_type = other DNA
gattgccttcacgaaa

SEQ ID NO: 375 - DNA, 14 bp, influenza B virus
  source 1..14: mol_type = other DNA
gccttcattttgtg

SEQ ID NO: 376 - DNA, 16 bp, influenza B virus
  source 1..16: mol_type = other DNA
attgccttcattttgt

SEQ ID NO: 377 - DNA, 16 bp, influenza B virus
  source 1..16: mol_type = other DNA
attgccttcattttgt

SEQ ID NO: 378 - DNA, 16 bp, influenza B virus
  source 1..16: mol_type = other DNA
tagtacaattattgcc

SEQ ID NO: 379 - DNA, 15 bp, influenza B virus
  source 1..15: mol_type = other DNA
agtacaattattgcc

SEQ ID NO: 380 - DNA, 16 bp, influenza B virus
  source 1..16: mol_type = other DNA
gtacaattattgcctt

SEQ ID NO: 381 - DNA, 15 bp, influenza B virus
  source 1..15: mol_type = other DNA
accatgagtagtaca

SEQ ID NO: 382 - DNA, 15 bp, influenza B virus
  source 1..15: mol_type = other DNA
catgagtagtacaat

SEQ ID NO: 383 - DNA, 17 bp, influenza B virus
  source 1..17: mol_type = other DNA
gatgttactaccatgag

SEQ ID NO: 384 - DNA, 16 bp, influenza B virus
  source 1..16: mol_type = other DNA
atgttactaccatgag

SEQ ID NO: 385 - DNA, 16 bp, influenza B virus
  source 1..16: mol_type = other DNA
cattggatgttactac

SEQ ID NO: 386 - DNA, 16 bp, influenza B virus
  source 1..16: mol_type = other DNA
attggatgttactacc

SEQ ID NO: 387 - DNA, 15 bp, influenza B virus
  source 1..15: mol_type = other DNA
attggatgttactac

SEQ ID NO: 388 - DNA, 16 bp, influenza B virus
  source 1..16: mol_type = other DNA
tttcgtgaaggcaatc

SEQ ID NO: 389 - DNA, 14 bp, influenza B virus
  source 1..14: mol_type = other DNA
tcgtgaaggcaatc

SEQ ID NO: 390 - DNA, 15 bp, synthetic construct
  misc_feature 1..15: note = synthetic sequence
  source 1..15: mol_type = other DNA
ggtttcgtccgtgtt

SEQ ID NO: 391 - DNA, 14 bp, synthetic construct
  misc_feature 1..14: note = synthetic sequence
  source 1..14: mol_type = other DNA
gtttcgtccgtgtt

SEQ ID NO: 392 - DNA, 15 bp, synthetic construct
  misc_feature 1..15: note = synthetic sequence
  source 1..15: mol_type = other DNA
gctgtcgcccgtgtc

SEQ ID NO: 393 - DNA, 15 bp, synthetic construct
  misc_feature 1..15: note = synthetic sequence
  source 1..15: mol_type = other DNA
gctgtcgcccgtgtc

SEQ ID NO: 394 - DNA, 15 bp, synthetic construct
  misc_feature 1..15: note = synthetic sequence
  source 1..15: mol_type = other DNA
gctgtcgcccgtgtc

SEQ ID NO: 395 - DNA, 14 bp, synthetic construct
  misc_feature 1..14: note = synthetic sequence
  source 1..14: mol_type = other DNA
gctgtcgcccgtgt

SEQ ID NO: 396 - DNA, 10 bp, synthetic construct
  misc_feature 1..10: note = synthetic sequence
  source 1..10: mol_type = other DNA
ttcgtccgtg

SEQ ID NO: 397 - DNA, 10 bp, synthetic construct
  misc_feature 1..10: note = synthetic sequence
  source 1..10: mol_type = other DNA
ttcgtccgtg

SEQ ID NO: 398 - DNA, 10 bp, synthetic construct
  misc_feature 1..10: note = synthetic sequence
  source 1..10: mol_type = other DNA
ttcgtccgtg

SEQ ID NO: 399-401 - skipped (3 entries)

SEQ ID NO: 402 - DNA, 10 bp, synthetic construct
  misc_feature 1..10: note = synthetic sequence
  source 1..10: mol_type = other DNA
tttcgtccgt

SEQ ID NO: 403 - DNA, 10 bp, synthetic construct
  misc_feature 1..10: note = synthetic sequence
  source 1..10: mol_type = other DNA
tttcgtccgt

SEQ ID NO: 404 - DNA, 10 bp, synthetic construct
  misc_feature 1..10: note = synthetic sequence
  source 1..10: mol_type = other DNA
tttcgtccgt

SEQ ID NO: 405 - DNA, 10 bp, synthetic construct
  misc_feature 1..10: note = synthetic sequence
  source 1..10: mol_type = other DNA
ccccacccac

SEQ ID NO: 406 - DNA, 10 bp, synthetic construct
  misc_feature 1..10: note = synthetic sequence
  source 1..10: mol_type = other DNA
ccccacccac

SEQ ID NO: 407 - DNA, 10 bp, synthetic construct
  misc_feature 1..10: note = synthetic sequence
  source 1..10: mol_type = other DNA
ccccacccac

SEQ ID NO: 408 - DNA, 12 bp, synthetic construct
  misc_feature 1..12: note = synthetic sequence
  source 1..12: mol_type = other DNA
tttcgtccgtgt

SEQ ID NO: 409 - DNA, 12 bp, synthetic construct
  misc_feature 1..12: note = synthetic sequence
  source 1..12: mol_type = other DNA
tttcgtccgtgt

SEQ ID NO: 410 - DNA, 12 bp, synthetic construct
  misc_feature 1..12: note = synthetic sequence
  source 1..12: mol_type = other DNA
tttcgtccgtgt

SEQ ID NO: 411 - DNA, 12 bp, synthetic construct
  misc_feature 1..12: note = synthetic sequence
  source 1..12: mol_type = other DNA
ttccatccatgt

SEQ ID NO: 412 - DNA, 12 bp, synthetic construct
  misc_feature 1..12: note = synthetic sequence
  source 1..12: mol_type = other DNA
ttccatccatgt

SEQ ID NO: 413 - DNA, 12 bp, synthetic construct
  misc_feature 1..12: note = synthetic sequence
  source 1..12: mol_type = other DNA
ttccatccatgt

SEQ ID NO: 414 - DNA, 12 bp, synthetic construct
  misc_feature 1..12: note = synthetic sequence
  source 1..12: mol_type = other DNA
ttccatccatgt

SEQ ID NO: 415 - DNA, 14 bp, synthetic construct
  misc_feature 1..14: note = synthetic sequence
  source 1..14: mol_type = other DNA
gtttcgtccgtgtt

SEQ ID NO: 416 - DNA, 14 bp, synthetic construct
  misc_feature 1..14: note = synthetic sequence
  source 1..14: mol_type = other DNA
gtttcgtccgtgtt

SEQ ID NO: 417 - DNA, 14 bp, synthetic construct
  misc_feature 1..14: note = synthetic sequence
  source 1..14: mol_type = other DNA
gtttcgtccgtgtt

SEQ ID NO: 418 - DNA, 14 bp, synthetic construct
  misc_feature 1..14: note = synthetic sequence
  source 1..14: mol_type = other DNA
gtttcggccatgtg

SEQ ID NO: 419 - DNA, 10 bp, synthetic construct
  misc_feature 1..10: note = synthetic sequence
  source 1..10: mol_type = other DNA
cgtccgtgtt

SEQ ID NO: 420 - DNA, 10 bp, synthetic construct
  misc_feature 1..10: note = synthetic sequence
  source 1..10: mol_type = other DNA
cgtccgtgtt

SEQ ID NO: 421 - DNA, 10 bp, synthetic construct
  misc_feature 1..10: note = synthetic sequence
  source 1..10: mol_type = other DNA
cgtccgtgtt

SEQ ID NO: 422 - DNA, 10 bp, synthetic construct
  misc_feature 1..10: note = synthetic sequence
  source 1..10: mol_type = other DNA
cgtccgtgtt

SEQ ID NO: 423 - DNA, 10 bp, synthetic construct
  misc_feature 1..10: note = synthetic sequence
  source 1..10: mol_type = other DNA
cctccgtgtc

SEQ ID NO: 424 - DNA, 10 bp, synthetic construct
  misc_feature 1..10: note = synthetic sequence
  source 1..10: mol_type = other DNA
cctccgtgtc

SEQ ID NO: 425 - DNA, 10 bp, synthetic construct
  misc_feature 1..10: note = synthetic sequence
  source 1..10: mol_type = other DNA
cctccgtgtc

SEQ ID NO: 426 - DNA, 10 bp, synthetic construct
  misc_feature 1..10: note = synthetic sequence
  source 1..10: mol_type = other DNA
tccgtgttgc

SEQ ID NO: 427 - DNA, 10 bp, synthetic construct
  misc_feature 1..10: note = synthetic sequence
  source 1..10: mol_type = other DNA
tccgtgttgc

SEQ ID NO: 428 - DNA, 10 bp, synthetic construct
  misc_feature 1..10: note = synthetic sequence
  source 1..10: mol_type = other DNA
tccgtgttgc

SEQ ID NO: 429 - DNA, 10 bp, synthetic construct
  misc_feature 1..10: note = synthetic sequence
  source 1..10: mol_type = other DNA
tccgtcttgc

SEQ ID NO: 430 - DNA, 13 bp, synthetic construct
  misc_feature 1..13: note = synthetic sequence
  misc_feature 13: note = n is a, c, g, or t
  source 1..13: mol_type = other DNA
tccgtcttgcsdn

SEQ ID NO: 431 - skipped

SEQ ID NO: 432 - DNA, 13 bp, synthetic construct
  misc_feature 1..13: note = synthetic sequence
  source 1..13: mol_type = other DNA
tttcgtccgtgtt

SEQ ID NO: 433 - DNA, 13 bp, synthetic construct
  misc_feature 1..13: note = synthetic sequence
  source 1..13: mol_type = other DNA
tttcgtccgtgtt

SEQ ID NO: 434 - DNA, 13 bp, synthetic construct
  misc_feature 1..13: note = synthetic sequence
  source 1..13: mol_type = other DNA
tttcctctatgtt

SEQ ID NO: 435 - DNA, 13 bp, synthetic construct
  misc_feature 1..13: note = synthetic sequence
  source 1..13: mol_type = other DNA
tttcctctatgtt

SEQ ID NO: 436 - DNA, 13 bp, synthetic construct
  misc_feature 1..13: note = synthetic sequence
  source 1..13: mol_type = other DNA
gtttcgtccgtgt

SEQ ID NO: 437 - DNA, 15 bp, synthetic construct
  misc_feature 1..15: note = synthetic sequence
  source 1..15: mol_type = other DNA
ggtttcgtccgtgtt

SEQ ID NO: 438 - DNA, 15 bp, synthetic construct
  misc_feature 1..15: note = synthetic sequence
  source 1..15: mol_type = other DNA
ggtttcgtccgtgtt

SEQ ID NO: 439 - DNA, 15 bp, synthetic construct
  misc_feature 1..15: note = synthetic sequence
  source 1..15: mol_type = other DNA
aagtacgtcctactt

SEQ ID NO: 440 - DNA, 10 bp, synthetic construct
  misc_feature 1..10: note = synthetic sequence
  source 1..10: mol_type = other DNA
ggtttcgtcc

SEQ ID NO: 441 - DNA, 10 bp, synthetic construct
  misc_feature 1..10: note = synthetic sequence
  source 1..10: mol_type = other DNA
ggtttcgtcc

SEQ ID NO: 442 - DNA, 15 bp, synthetic construct
  misc_feature 1..15: note = synthetic sequence
  source 1..15: mol_type = other DNA
tgggtttcgtccgtt

SEQ ID NO: 443 - DNA, 14 bp, synthetic construct
  misc_feature 1..14: note = synthetic sequence
  source 1..14: mol_type = other DNA
ttttgggattccgt

SEQ ID NO: 444 - DNA, 16 bp, synthetic construct
  misc_feature 1..16: note = synthetic sequence
  source 1..16: mol_type = other DNA
gcttttgggattccgt

SEQ ID NO: 445 - DNA, 16 bp, synthetic construct
  misc_feature 1..16: note = synthetic sequence
  source 1..16: mol_type = other DNA
gcttttgggattccgt

SEQ ID NO: 446 - DNA, 16 bp, synthetic construct
  misc_feature 1..16: note = synthetic sequence
  source 1..16: mol_type = other DNA
agctgcttttgggatt

SEQ ID NO: 447 - DNA, 16 bp, synthetic construct
  misc_feature 1..16: note = synthetic sequence
  source 1..16: mol_type = other DNA
gagctgcttttgggat

SEQ ID NO: 448 - DNA, 16 bp, synthetic construct
  misc_feature 1..16: note = synthetic sequence
  source 1..16: mol_type = other DNA
ctgcttttgggattcc

SEQ ID NO: 449 - DNA, 14 bp, synthetic construct
  misc_feature 1..14: note = synthetic sequence
  source 1..14: mol_type = other DNA
tgcttttgggattc

SEQ ID NO: 450 - DNA, 16 bp, synthetic construct
  misc_feature 1..16: note = synthetic sequence
  source 1..16: mol_type = other DNA
agctgcttttgggatt

SEQ ID NO: 451 - DNA, 14 bp, synthetic construct
  misc_feature 1..14: note = synthetic sequence
  source 1..14: mol_type = other DNA
agctgcttttggga

SEQ ID NO: 452 - DNA, 16 bp, synthetic construct
  misc_feature 1..16: note = synthetic sequence
  source 1..16: mol_type = other DNA
cagctgcttttgggat

SEQ ID NO: 453 - DNA, 16 bp, synthetic construct
  misc_feature 1..16: note = synthetic sequence
  source 1..16: mol_type = other DNA
agctgcttttgggatt

SEQ ID NO: 454 - DNA, 14 bp, synthetic construct
  misc_feature 1..14: note = synthetic sequence
  source 1..14: mol_type = other DNA
agctgcttttggga

SEQ ID NO: 455 - DNA, 14 bp, synthetic construct
  misc_feature 1..14: note = synthetic sequence
  source 1..14: mol_type = other DNA
agctgcttttggga

SEQ ID NO: 456 - DNA, 16 bp, synthetic construct
  misc_feature 1..16: note = synthetic sequence
  source 1..16: mol_type = other DNA
agctgcttttgggatt

SEQ ID NO: 457 - DNA, 14 bp, synthetic construct
  misc_feature 1..14: note = synthetic sequence
  source 1..14: mol_type = other DNA
tgcttttgggattc

SEQ ID NO: 458 - DNA, 14 bp, synthetic construct
  misc_feature 1..14: note = synthetic sequence
  source 1..14: mol_type = other DNA
gcggcgccccgcct

SEQ ID NO: 459 - DNA, 14 bp, synthetic construct
  misc_feature 1..14: note = synthetic sequence
  source 1..14: mol_type = other DNA
gcggcgccccgcct

SEQ ID NO: 460 - DNA, 21 bp, synthetic construct
  misc_feature 1..21: note = synthetic sequence
  source 1..21: mol_type = other DNA
cggtcccgcggcgccccgcct

SEQ ID NO: 461 - DNA, 16 bp, synthetic construct
  misc_feature 1..16: note = synthetic sequence
  source 1..16: mol_type = other DNA
tttgggcttcctcgct

SEQ ID NO: 462 - DNA, 14 bp, synthetic construct
  misc_feature 1..14: note = synthetic sequence
  source 1..14: mol_type = other DNA
tttgggcttcctcg

SEQ ID NO: 463 - DNA, 14 bp, synthetic construct
  misc_feature 1..14: note = synthetic sequence
  source 1..14: mol_type = other DNA
tttgggcttcctcg

SEQ ID NO: 464 - DNA, 14 bp, synthetic construct
  misc_feature 1..14: note = synthetic sequence
  source 1..14: mol_type = other DNA
tgggcttcctcgct

SEQ ID NO: 465 - DNA, 16 bp, synthetic construct
  misc_feature 1..16: note = synthetic sequence
  source 1..16: mol_type = other DNA
atatactttgggcttc

SEQ ID NO: 466 - DNA, 16 bp, synthetic construct
  misc_feature 1..16: note = synthetic sequence
  source 1..16: mol_type = other DNA
atatactttgggcttc

SEQ ID NO: 467 - DNA, 14 bp, synthetic construct
  misc_feature 1..14: note = synthetic sequence
  source 1..14: mol_type = other DNA
atatactttgggct

SEQ ID NO: 468 - DNA, 15 bp, synthetic construct
  misc_feature 1..15: note = synthetic sequence
  source 1..15: mol_type = other DNA
atatactttgggctt

SEQ ID NO: 469 - DNA, 16 bp, synthetic construct
  misc_feature 1..16: note = synthetic sequence
  source 1..16: mol_type = other DNA
tagccctagccccgca

SEQ ID NO: 470 - DNA, 16 bp, synthetic construct
  misc_feature 1..16: note = synthetic sequence
  source 1..16: mol_type = other DNA
tagccctagccccgca

SEQ ID NO: 471 - DNA, 14 bp, synthetic construct
  misc_feature 1..14: note = synthetic sequence
  source 1..14: mol_type = other DNA
tagccctagccccg

SEQ ID NO: 472 - DNA, 14 bp, synthetic construct
  misc_feature 1..14: note = synthetic sequence
  source 1..14: mol_type = other DNA
tgctgttagcccta

SEQ ID NO: 473 - DNA, 14 bp, synthetic construct
  misc_feature 1..14: note = synthetic sequence
  source 1..14: mol_type = other DNA
tgctgttagcccta

SEQ ID NO: 474 - DNA, 15 bp, synthetic construct
  misc_feature 1..15: note = synthetic sequence
  source 1..15: mol_type = other DNA
gtgttagccctagcc

SEQ ID NO: 475 - DNA, 14 bp, synthetic construct
  misc_feature 1..14: note = synthetic sequence
  source 1..14: mol_type = other DNA
gcgcccagccccgc

SEQ ID NO: 476 - DNA, 14 bp, synthetic construct
  misc_feature 1..14: note = synthetic sequence
  source 1..14: mol_type = other DNA
gcgcccagccccgc

SEQ ID NO: 477 - DNA, 14 bp, synthetic construct
  misc_feature 1..14: note = synthetic sequence
  source 1..14: mol_type = other DNA
cgcgcgcccagccc

SEQ ID NO: 478 - DNA, 17 bp, synthetic construct
  misc_feature 1..17: note = synthetic sequence
  source 1..17: mol_type = other DNA
cgcgcgcccagccccgc

SEQ ID NO: 479 - DNA, 14 bp, synthetic construct
  misc_feature 1..14: note = synthetic sequence
  source 1..14: mol_type = other DNA
tggcatggaatggg

SEQ ID NO: 480 - DNA, 16 bp, synthetic construct
  misc_feature 1..16: note = synthetic sequence
  source 1..16: mol_type = other DNA
atggaatgggctccgc

SEQ ID NO: 481 - DNA, 14 bp, synthetic construct
  misc_feature 1..14: note = synthetic sequence
  source 1..14: mol_type = other DNA
atggaatgggctcc

SEQ ID NO: 482 - DNA, 15 bp, synthetic construct
  misc_feature 1..15: note = synthetic sequence
  source 1..15: mol_type = other DNA
aatgggctccgccag

SEQ ID NO: 483 - DNA, 15 bp, synthetic construct
  misc_feature 1..15: note = synthetic sequence
  source 1..15: mol_type = other DNA
aatgggctccgccag

SEQ ID NO: 484 - DNA, 14 bp, synthetic construct
  misc_feature 1..14: note = synthetic sequence
  source 1..14: mol_type = other DNA
aatgggctccgcca

SEQ ID NO: 485 - DNA, 14 bp, synthetic construct
  misc_feature 1..14: note = synthetic sequence
  source 1..14: mol_type = other DNA
aatgggctccgcca

SEQ ID NO: 486 - DNA, 16 bp, synthetic construct
  misc_feature 1..16: note = synthetic sequence
  source 1..16: mol_type = other DNA
cttacccgaggcggtc

SEQ ID NO: 487 - DNA, 14 bp, synthetic construct
  misc_feature 1..14: note = synthetic sequence
  source 1..14: mol_type = other DNA
ttacccgaggcggt

SEQ ID NO: 488 - DNA, 16 bp, synthetic construct
  misc_feature 1..16: note = synthetic sequence
  source 1..16: mol_type = other DNA
accgtaccttacccga

SEQ ID NO: 489 - DNA, 14 bp, synthetic construct
  misc_feature 1..14: note = synthetic sequence
  source 1..14: mol_type = other DNA
cgtaccttacccga

SEQ ID NO: 490 - DNA, 14 bp, synthetic construct
  misc_feature 1..14: note = synthetic sequence
  source 1..14: mol_type = other DNA
ctccgagccccgcc

SEQ ID NO: 491 - DNA, 19 bp, synthetic construct
  misc_feature 1..19: note = synthetic sequence
  source 1..19: mol_type = other DNA
cccggctccgagccccgcc

SEQ ID NO: 492 - DNA, 15 bp, synthetic construct
  misc_feature 1..15: note = synthetic sequence
  source 1..15: mol_type = other DNA
tggcctgtccccgca

SEQ ID NO: 493 - DNA, 15 bp, synthetic construct
  misc_feature 1..15: note = synthetic sequence
  source 1..15: mol_type = other DNA
tggcctgtccccgca

SEQ ID NO: 494 - DNA, 14 bp, synthetic construct
  misc_feature 1..14: note = synthetic sequence
  source 1..14: mol_type = other DNA
gatgccctggcctg

SEQ ID NO: 495 - DNA, 14 bp, synthetic construct
  misc_feature 1..14: note = synthetic sequence
  source 1..14: mol_type = other DNA
gatgccctggcctg

SEQ ID NO: 496 - DNA, 14 bp, synthetic construct
  misc_feature 1..14: note = synthetic sequence
  source 1..14: mol_type = other DNA
gcagccagctctac

SEQ ID NO: 497 - DNA, 14 bp, synthetic construct
  misc_feature 1..14: note = synthetic sequence
  source 1..14: mol_type = other DNA
gcagccagctctac

SEQ ID NO: 498 - DNA, 14 bp, synthetic construct
  misc_feature 1..14: note = synthetic sequence
  source 1..14: mol_type = other DNA
agccagctctaccc

SEQ ID NO: 499 - DNA, 16 bp, synthetic construct
  misc_feature 1..16: note = synthetic sequence
  source 1..16: mol_type = other DNA
agctctacccccgcca

SEQ ID NO: 500 - DNA, 16 bp, synthetic construct
  misc_feature 1..16: note = synthetic sequence
  source 1..16: mol_type = other DNA
agctctacccccgcca

SEQ ID NO: 501 - DNA, 16 bp, synthetic construct
  misc_feature 1..16: note = synthetic sequence
  source 1..16: mol_type = other DNA
aaagcagcgcccactt

SEQ ID NO: 502 - DNA, 14 bp, synthetic construct
  misc_feature 1..14: note = synthetic sequence
  source 1..14: mol_type = other DNA
acttcctccccgct

SEQ ID NO: 503 - DNA, 16 bp, synthetic construct
  misc_feature 1..16: note = synthetic sequence
  source 1..16: mol_type = other DNA
ctacagaagccccata

SEQ ID NO: 504 - DNA, 16 bp, synthetic construct
  misc_feature 1..16: note = synthetic sequence
  source 1..16: mol_type = other DNA
ctacagaagccccata

SEQ ID NO: 505 - DNA, 16 bp, synthetic construct
  misc_feature 1..16: note = synthetic sequence
  source 1..16: mol_type = other DNA
gaaatctctacagaag

SEQ ID NO: 506 - DNA, 16 bp, synthetic construct
  misc_feature 1..16: note = synthetic sequence
  source 1..16: mol_type = other DNA
gaaatctctacagaag

SEQ ID NO: 507 - DNA, 16 bp, synthetic construct
  misc_feature 1..16: note = synthetic sequence
  source 1..16: mol_type = other DNA
tgatccctgtccccat

SEQ ID NO: 508 - DNA, 15 bp, synthetic construct
  misc_feature 1..15: note = synthetic sequence
  source 1..15: mol_type = other DNA
atgctgatccctgtc

SEQ ID NO: 509 - DNA, 23 bp, synthetic construct
  misc_feature 1..23: note = synthetic sequence
  source 1..23: mol_type = other DNA
gccatgctgatccctgtccccat

SEQ ID NO: 510 - DNA, 14 bp, synthetic construct
  misc_feature 1..14: note = synthetic sequence
  source 1..14: mol_type = other DNA
ccatctcaccccat

SEQ ID NO: 511 - DNA, 15 bp, synthetic construct
  misc_feature 1..15: note = synthetic sequence
  source 1..15: mol_type = other DNA
gctgctcctccccat

SEQ ID NO: 512 - DNA, 15 bp, synthetic construct
  misc_feature 1..15: note = synthetic sequence
  source 1..15: mol_type = other DNA
tctccaaccccacaa

SEQ ID NO: 513 - DNA, 14 bp, synthetic construct
  misc_feature 1..14: note = synthetic sequence
  source 1..14: mol_type = other DNA
ctccaaccccacaa

SEQ ID NO: 514 - DNA, 15 bp, synthetic construct
  misc_feature 1..15: note = synthetic sequence
  source 1..15: mol_type = other DNA
cagccagctctccaa

SEQ ID NO: 515 - DNA, 14 bp, synthetic construct
  misc_feature 1..14: note = synthetic sequence
  source 1..14: mol_type = other DNA
agccagctctccaa

SEQ ID NO: 516 - DNA, 17 bp, synthetic construct
  misc_feature 1..17: note = synthetic sequence
  source 1..17: mol_type = other DNA
atctgttctctaaacga

SEQ ID NO: 517 - DNA, 16 bp, synthetic construct
  misc_feature 1..16: note = synthetic sequence
  source 1..16: mol_type = other DNA
atctgttctctaaacg

SEQ ID NO: 518 - DNA, 16 bp, synthetic construct
  misc_feature 1..16: note = synthetic sequence
  source 1..16: mol_type = other DNA
agatctgttctctaaa

SEQ ID NO: 519 - DNA, 16 bp, synthetic construct
  misc_feature 1..16: note = synthetic sequence
  source 1..16: mol_type = other DNA
tctctaaacgaacttt

SEQ ID NO: 520 - DNA, 16 bp, synthetic construct
  misc_feature 1..16: note = synthetic sequence
  source 1..16: mol_type = other DNA
tctctaaacgaacttt

SEQ ID NO: 521 - DNA, 16 bp, synthetic construct
  misc_feature 1..16: note = synthetic sequence
  source 1..16: mol_type = other DNA
ctctaaacgaacttta

SEQ ID NO: 522 - DNA, 14 bp, synthetic construct
  misc_feature 1..14: note = synthetic sequence
  source 1..14: mol_type = other DNA
actttaaaatctgt

SEQ ID NO: 523 - DNA, 15 bp, synthetic construct
  misc_feature 1..15: note = synthetic sequence
  source 1..15: mol_type = other DNA
ggtttcgtccgtgtt

SEQ ID NO: 524 - DNA, 15 bp, synthetic construct
  misc_feature 1..15: note = synthetic sequence
  source 1..15: mol_type = other DNA
ggtttcgtccgtgtt

SEQ ID NO: 525 - DNA, 15 bp, synthetic construct
  misc_feature 1..15: note = synthetic sequence
  source 1..15: mol_type = other DNA
ggtttcgtccgtgtt

SEQ ID NO: 526 - DNA, 17 bp, synthetic construct
  misc_feature 1..17: note = synthetic sequence
  source 1..17: mol_type = other DNA
tgcttacggtttcgtcc

SEQ ID NO: 527 - DNA, 16 bp, synthetic construct
  misc_feature 1..16: note = synthetic sequence
  source 1..16: mol_type = other DNA
gtttcgtccgtgttgc

SEQ ID NO: 528 - DNA, 14 bp, synthetic construct
  misc_feature 1..14: note = synthetic sequence
  source 1..14: mol_type = other DNA
taggtttcgtccgg

SEQ ID NO: 529 - DNA, 14 bp, synthetic construct
  misc_feature 1..14: note = synthetic sequence
  source 1..14: mol_type = other DNA
tcgtccgggtgtga

SEQ ID NO: 530 - DNA, 15 bp, synthetic construct
  misc_feature 1..15: note = synthetic sequence
  source 1..15: mol_type = other DNA
ttcgtccgggtgtga

SEQ ID NO: 531 - DNA, 16 bp, synthetic construct
  misc_feature 1..16: note = synthetic sequence
  source 1..16: mol_type = other DNA
tttcgtccgggtgtga

SEQ ID NO: 532 - DNA, 15 bp, synthetic construct
  misc_feature 1..15: note = synthetic sequence
  source 1..15: mol_type = other DNA
aggtttcgtccgggt

SEQ ID NO: 533 - DNA, 14 bp, synthetic construct
  misc_feature 1..14: note = synthetic sequence
  source 1..14: mol_type = other DNA
aggtttcgtccggg

SEQ ID NO: 534 - DNA, 15 bp, synthetic construct
  misc_feature 1..15: note = synthetic sequence
  source 1..15: mol_type = other DNA
aggtttcgtccgggt

SEQ ID NO: 535 - DNA, 15 bp, synthetic construct
  misc_feature 1..15: note = synthetic sequence
  source 1..15: mol_type = other DNA
tttcgtccgggtgtg

SEQ ID NO: 536 - DNA, 15 bp, synthetic construct
  misc_feature 1..15: note = synthetic sequence
  source 1..15: mol_type = other DNA
aggccacgcggagta

SEQ ID NO: 537 - DNA, 16 bp, synthetic construct
  misc_feature 1..16: note = synthetic sequence
  source 1..16: mol_type = other DNA
cacgcggagtacgatc

SEQ ID NO: 538 - DNA, 14 bp, synthetic construct
  misc_feature 1..14: note = synthetic sequence
  source 1..14: mol_type = other DNA
tgtcagtaagtatg

SEQ ID NO: 539 - DNA, 16 bp, synthetic construct
  misc_feature 1..16: note = synthetic sequence
  source 1..16: mol_type = other DNA
ctggctgtcagtaagt

SEQ ID NO: 540 - DNA, 15 bp, synthetic construct
  misc_feature 1..15: note = synthetic sequence
  source 1..15: mol_type = other DNA
tcgctgtctggctgt

SEQ ID NO: 541 - DNA, 16 bp, synthetic construct
  misc_feature 1..16: note = synthetic sequence
  source 1..16: mol_type = other DNA
cttttggtcgctgtct

SEQ ID NO: 542 - DNA, 14 bp, synthetic construct
  misc_feature 1..14: note = synthetic sequence
  source 1..14: mol_type = other DNA
cttttggtcgctgt

SEQ ID NO: 543 - DNA, 16 bp, synthetic construct
  misc_feature 1..16: note = synthetic sequence
  source 1..16: mol_type = other DNA
ttggtcgctgtctggc

SEQ ID NO: 544 - DNA, 14 bp, synthetic construct
  misc_feature 1..14: note = synthetic sequence
  source 1..14: mol_type = other DNA
ttggtcgctgtctg

SEQ ID NO: 545 - DNA, 16 bp, synthetic construct
  misc_feature 1..16: note = synthetic sequence
  source 1..16: mol_type = other DNA
gaattcttttggtcgc

SEQ ID NO: 546 - DNA, 15 bp, synthetic construct
  misc_feature 1..15: note = synthetic sequence
  source 1..15: mol_type = other DNA
gaattcttttggtcg

SEQ ID NO: 547 - DNA, 15 bp, synthetic construct
  misc_feature 1..15: note = synthetic sequence
  source 1..15: mol_type = other DNA
aattcttttggtcgc

SEQ ID NO: 548 - DNA, 16 bp, synthetic construct
  misc_feature 1..16: note = synthetic sequence
  source 1..16: mol_type = other DNA
cgaattcttttggtcg

SEQ ID NO: 549 - DNA, 15 bp, synthetic construct
  misc_feature 1..15: note = synthetic sequence
  source 1..15: mol_type = other DNA
acactaattgatggc

SEQ ID NO: 550 - DNA, 13 bp, synthetic construct
  misc_feature 1..13: note = synthetic sequence
  source 1..13: mol_type = other DNA
aattgatggccat

SEQ ID NO: 551 - DNA, 16 bp, synthetic construct
  misc_feature 1..16: note = synthetic sequence
  source 1..16: mol_type = other DNA
ccacaaaatgaaggca

SEQ ID NO: 552 - DNA, 15 bp, synthetic construct
  misc_feature 1..15: note = synthetic sequence
  source 1..15: mol_type = other DNA
cacaaaatgaaggca

SEQ ID NO: 553 - DNA, 15 bp, synthetic construct
  misc_feature 1..15: note = synthetic sequence
  source 1..15: mol_type = other DNA
cacaaaatgaaggca

SEQ ID NO: 554 - DNA, 14 bp, synthetic construct
  misc_feature 1..14: note = synthetic sequence
  source 1..14: mol_type = other DNA
cacaaaatgaaggc

SEQ ID NO: 555 - DNA, 14 bp, synthetic construct
  misc_feature 1..14: note = synthetic sequence
  source 1..14: mol_type = other DNA
caataattgtacta

SEQ ID NO: 556 - DNA, 14 bp, synthetic construct
  misc_feature 1..14: note = synthetic sequence
  source 1..14: mol_type = other DNA
caataattgtacta

SEQ ID NO: 557 - DNA, 14 bp, synthetic construct
  misc_feature 1..14: note = synthetic sequence
  source 1..14: mol_type = other DNA
caataattgtacta

SEQ ID NO: 558 - DNA, 15 bp, synthetic construct
  misc_feature 1..15: note = synthetic sequence
  source 1..15: mol_type = other DNA
caataattgtactac

SEQ ID NO: 559 - DNA, 15 bp, synthetic construct
  misc_feature 1..15: note = synthetic sequence
  source 1..15: mol_type = other DNA
caataattgtactac

SEQ ID NO: 560 - DNA, 16 bp, synthetic construct
  misc_feature 1..16: note = synthetic sequence
  source 1..16: mol_type = other DNA
tgtactactcatggta

SEQ ID NO: 561 - DNA, 16 bp, synthetic construct
  misc_feature 1..16: note = synthetic sequence
  source 1..16: mol_type = other DNA
tgtactactcatggta

SEQ ID NO: 562 - DNA, 16 bp, synthetic construct
  misc_feature 1..16: note = synthetic sequence
  source 1..16: mol_type = other DNA
tgtactactcatggta

SEQ ID NO: 563 - DNA, 14 bp, synthetic construct
  misc_feature 1..14: note = synthetic sequence
  source 1..14: mol_type = other DNA
gtactactcatggt

SEQ ID NO: 564 - DNA, 14 bp, synthetic construct
  misc_feature 1..14: note = synthetic sequence
  source 1..14: mol_type = other DNA
gtactactcatggt

SEQ ID NO: 565 - DNA, 15 bp, synthetic construct
  misc_feature 1..15: note = synthetic sequence
  source 1..15: mol_type = other DNA
ttgtactactcatgg

SEQ ID NO: 566 - DNA, 15 bp, synthetic construct
  misc_feature 1..15: note = synthetic sequence
  source 1..15: mol_type = other DNA
catggtagtaacatc

SEQ ID NO: 567 - DNA, 17 bp, synthetic construct
  misc_feature 1..17: note = synthetic sequence
  source 1..17: mol_type = other DNA
ctcatggtagtaacatc

SEQ ID NO: 568 - DNA, 16 bp, synthetic construct
  misc_feature 1..16: note = synthetic sequence
  source 1..16: mol_type = other DNA
ctcatggtagtaacat

SEQ ID NO: 569 - DNA, 16 bp, synthetic construct
  misc_feature 1..16: note = synthetic sequence
  source 1..16: mol_type = other DNA
ctcatggtagtaacat

SEQ ID NO: 570 - DNA, 16 bp, synthetic construct
  misc_feature 1..16: note = synthetic sequence
  source 1..16: mol_type = other DNA
actcatggtagtaaca

SEQ ID NO: 571 - DNA, 16 bp, synthetic construct
  misc_feature 1..16: note = synthetic sequence
  source 1..16: mol_type = other DNA
actcatggtagtaaca

SEQ ID NO: 572 - DNA, 15 bp, synthetic construct
  misc_feature 1..15: note = synthetic sequence
  source 1..15: mol_type = other DNA
actcatggtagtaac

SEQ ID NO: 573 - DNA, 14 bp, synthetic construct
  misc_feature 1..14: note = synthetic sequence
  source 1..14: mol_type = other DNA
actcatggtagtaa

SEQ ID NO: 574 - DNA, 15 bp, synthetic construct
  misc_feature 1..15: note = synthetic sequence
  source 1..15: mol_type = other DNA
caatgcagatcgaat

SEQ ID NO: 575 - DNA, 15 bp, synthetic construct
  misc_feature 1..15: note = synthetic sequence
  source 1..15: mol_type = other DNA
caatgcagatcgaat

SEQ ID NO: 576 - DNA, 16 bp, synthetic construct
  misc_feature 1..16: note = synthetic sequence
  source 1..16: mol_type = other DNA
gattgccttcacgaaa

SEQ ID NO: 577 - DNA, 16 bp, synthetic construct
  misc_feature 1..16: note = synthetic sequence
  source 1..16: mol_type = other DNA
gattgccttcacgaaa

SEQ ID NO: 578 - DNA, 14 bp, synthetic construct
  misc_feature 1..14: note = synthetic sequence
  source 1..14: mol_type = other DNA
gccttcattttgtg

SEQ ID NO: 579 - DNA, 16 bp, synthetic construct
  misc_feature 1..16: note = synthetic sequence
  source 1..16: mol_type = other DNA
attgccttcattttgt

SEQ ID NO: 580 - DNA, 16 bp, synthetic construct
  misc_feature 1..16: note = synthetic sequence
  source 1..16: mol_type = other DNA
attgccttcattttgt

SEQ ID NO: 581 - DNA, 16 bp, synthetic construct
  misc_feature 1..16: note = synthetic sequence
  source 1..16: mol_type = other DNA
tagtacaattattgcc

SEQ ID NO: 582 - DNA, 15 bp, synthetic construct
  misc_feature 1..15: note = synthetic sequence
  source 1..15: mol_type = other DNA
agtacaattattgcc

SEQ ID NO: 583 - DNA, 16 bp, synthetic construct
  misc_feature 1..16: note = synthetic sequence
  source 1..16: mol_type = other DNA
gtacaattattgcctt

SEQ ID NO: 584 - DNA, 15 bp, synthetic construct
  misc_feature 1..15: note = synthetic sequence
  source 1..15: mol_type = other DNA
accatgagtagtaca

SEQ ID NO: 585 - DNA, 15 bp, synthetic construct
  misc_feature 1..15: note = synthetic sequence
  source 1..15: mol_type = other DNA
catgagtagtacaat

SEQ ID NO: 586 - DNA, 17 bp, synthetic construct
  misc_feature 1..17: note = synthetic sequence
  source 1..17: mol_type = other DNA
gatgttactaccatgag

SEQ ID NO: 587 - DNA, 16 bp, synthetic construct
  misc_feature 1..16: note = synthetic sequence
  source 1..16: mol_type = other DNA
atgttactaccatgag

SEQ ID NO: 588 - DNA, 16 bp, synthetic construct
  misc_feature 1..16: note = synthetic sequence
  source 1..16: mol_type = other DNA
cattggatgttactac

SEQ ID NO: 589 - DNA, 16 bp, synthetic construct
  misc_feature 1..16: note = synthetic sequence
  source 1..16: mol_type = other DNA
attggatgttactacc

SEQ ID NO: 590 - DNA, 15 bp, synthetic construct
  misc_feature 1..15: note = synthetic sequence
  source 1..15: mol_type = other DNA
attggatgttactac

SEQ ID NO: 591 - DNA, 16 bp, synthetic construct
  misc_feature 1..16: note = synthetic sequence
  source 1..16: mol_type = other DNA
tttcgtgaaggcaatc

SEQ ID NO: 592 - DNA, 14 bp, synthetic construct
  misc_feature 1..14: note = synthetic sequence
  source 1..14: mol_type = other DNA
tcgtgaaggcaatc

SEQ ID NO: 593 - DNA, 17 bp, synthetic construct
  misc_feature 1..17: note = synthetic sequence
  source 1..17: mol_type = other DNA
atctgttctctaaacga

SEQ ID NO: 594 - DNA, 16 bp, synthetic construct
  misc_feature 1..16: note = synthetic sequence
  source 1..16: mol_type = other DNA
atctgttctctaaacg

SEQ ID NO: 595 - DNA, 16 bp, synthetic construct
  misc_feature 1..16: note = synthetic sequence
  source 1..16: mol_type = other DNA
agatctgttctctaaa

SEQ ID NO: 596 - DNA, 16 bp, synthetic construct
  misc_feature 1..16: note = synthetic sequence
  source 1..16: mol_type = other DNA
tctctaaacgaacttt

SEQ ID NO: 597 - DNA, 16 bp, synthetic construct
  misc_feature 1..16: note = synthetic sequence
  source 1..16: mol_type = other DNA
tctctaaacgaacttt

SEQ ID NO: 598 - DNA, 16 bp, synthetic construct
  misc_feature 1..16: note = synthetic sequence
  source 1..16: mol_type = other DNA
ctctaaacgaacttta

SEQ ID NO: 599 - DNA, 14 bp, synthetic construct
  misc_feature 1..14: note = synthetic sequence
  source 1..14: mol_type = other DNA
actttaaaatctgt

SEQ ID NO: 600 - DNA, 15 bp, synthetic construct
  misc_feature 1..15: note = synthetic sequence
  source 1..15: mol_type = other DNA
ggtttcgtccgtgtt

SEQ ID NO: 601 - DNA, 15 bp, synthetic construct
  misc_feature 1..15: note = synthetic sequence
  source 1..15: mol_type = other DNA
ggtttcgtccgtgtt

SEQ ID NO: 602 - DNA, 15 bp, synthetic construct
  misc_feature 1..15: note = synthetic sequence
  source 1..15: mol_type = other DNA
ggtttcgtccgtgtt

SEQ ID NO: 603 - DNA, 17 bp, synthetic construct
  misc_feature 1..17: note = synthetic sequence
  source 1..17: mol_type = other DNA
tgcttacggtttcgtcc

SEQ ID NO: 604 - DNA, 16 bp, synthetic construct
  misc_feature 1..16: note = synthetic sequence
  source 1..16: mol_type = other DNA
gtttcgtccgtgttgc

SEQ ID NO: 605 - DNA, 14 bp, synthetic construct
  misc_feature 1..14: note = synthetic sequence
  source 1..14: mol_type = other DNA
taggtttcgtccgg

SEQ ID NO: 606 - DNA, 14 bp, synthetic construct
  misc_feature 1..14: note = synthetic sequence
  source 1..14: mol_type = other DNA
tcgtccgggtgtga

SEQ ID NO: 607 - DNA, 15 bp, synthetic construct
  misc_feature 1..15: note = synthetic sequence
  source 1..15: mol_type = other DNA
ttcgtccgggtgtga

SEQ ID NO: 608 - DNA, 16 bp, synthetic construct
  misc_feature 1..16: note = synthetic sequence
  source 1..16: mol_type = other DNA
tttcgtccgggtgtga

SEQ ID NO: 609 - DNA, 15 bp, synthetic construct
  misc_feature 1..15: note = synthetic sequence
  source 1..15: mol_type = other DNA
aggtttcgtccgggt

SEQ ID NO: 610 - DNA, 14 bp, synthetic construct
  misc_feature 1..14: note = synthetic sequence
  source 1..14: mol_type = other DNA
aggtttcgtccggg

SEQ ID NO: 611 - DNA, 15 bp, synthetic construct
  misc_feature 1..15: note = synthetic sequence
  source 1..15: mol_type = other DNA
aggtttcgtccgggt

SEQ ID NO: 612 - DNA, 15 bp, synthetic construct
  misc_feature 1..15: note = synthetic sequence
  source 1..15: mol_type = other DNA
tttcgtccgggtgtg

SEQ ID NO: 613 - DNA, 15 bp, synthetic construct
  misc_feature 1..15: note = synthetic sequence
  source 1..15: mol_type = other DNA
aggccacgcggagta

SEQ ID NO: 614 - DNA, 16 bp, synthetic construct
  misc_feature 1..16: note = synthetic sequence
  source 1..16: mol_type = other DNA
cacgcggagtacgatc

SEQ ID NO: 615 - DNA, 15 bp, synthetic construct
  misc_feature 1..15: note = synthetic sequence
  source 1..15: mol_type = other DNA
gcggagtacgatcga

SEQ ID NO: 616 - DNA, 16 bp, synthetic construct
  misc_feature 1..16: note = synthetic sequence
  source 1..16: mol_type = other DNA
gcggagtacgatcgag

SEQ ID NO: 617 - DNA, 16 bp, synthetic construct
  misc_feature 1..16: note = synthetic sequence
  source 1..16: mol_type = other DNA
gcggagtacgatcgag

SEQ ID NO: 618 - DNA, 14 bp, synthetic construct
  misc_feature 1..14: note = synthetic sequence
  source 1..14: mol_type = other DNA
aggccacgcggagt

SEQ ID NO: 619 - DNA, 16 bp, synthetic construct
  misc_feature 1..16: note = synthetic sequence
  source 1..16: mol_type = other DNA
taactttaatctcaca

SEQ ID NO: 620 - DNA, 16 bp, synthetic construct
  misc_feature 1..16: note = synthetic sequence
  source 1..16: mol_type = other DNA
atctcacatagcaatc

SEQ ID NO: 621 - DNA, 16 bp, synthetic construct
  misc_feature 1..16: note = synthetic sequence
  source 1..16: mol_type = other DNA
cacatagcaatcttta

SEQ ID NO: 622 - DNA, 16 bp, synthetic construct
  misc_feature 1..16: note = synthetic sequence
  source 1..16: mol_type = other DNA
atagcaatctttaatc

SEQ ID NO: 623 - DNA, 17 bp, synthetic construct
  misc_feature 1..17: note = synthetic sequence
  source 1..17: mol_type = other DNA
gtagttaactttaatct

SEQ ID NO: 624 - DNA, 16 bp, synthetic construct
  misc_feature 1..16: note = synthetic sequence
  source 1..16: mol_type = other DNA
taactttaatctcaca

SEQ ID NO: 625 - DNA, 16 bp, synthetic construct
  misc_feature 1..16: note = synthetic sequence
  source 1..16: mol_type = other DNA
taactttaatctcaca

SEQ ID NO: 626 - DNA, 17 bp, synthetic construct
  misc_feature 1..17: note = synthetic sequence
  source 1..17: mol_type = other DNA
ctttaatctcacatagc

SEQ ID NO: 627 - DNA, 14 bp, synthetic construct
  misc_feature 1..14: note = synthetic sequence
  source 1..14: mol_type = other DNA
cacatagcaatctt

SEQ ID NO: 628 - DNA, 16 bp, synthetic construct
  misc_feature 1..16: note = synthetic sequence
  source 1..16: mol_type = other DNA
ctcacatagcaatctt

SEQ ID NO: 629 - DNA, 16 bp, synthetic construct
  misc_feature 1..16: note = synthetic sequence
  source 1..16: mol_type = other DNA
cgtgctacaacttcct

SEQ ID NO: 630 - DNA, 15 bp, synthetic construct
  misc_feature 1..15: note = synthetic sequence
  source 1..15: mol_type = other DNA
tgctacaacttcctc

SEQ ID NO: 631 - DNA, 16 bp, synthetic construct
  misc_feature 1..16: note = synthetic sequence
  source 1..16: mol_type = other DNA
ctcaaggaacaacatt

SEQ ID NO: 632 - DNA, 15 bp, synthetic construct
  misc_feature 1..15: note = synthetic sequence
  source 1..15: mol_type = other DNA
aaggcttctacgcag

SEQ ID NO: 633 - DNA, 15 bp, synthetic construct
  misc_feature 1..15: note = synthetic sequence
  source 1..15: mol_type = other DNA
tgctacaacttcctc

SEQ ID NO: 634 - DNA, 14 bp, synthetic construct
  misc_feature 1..14: note = synthetic sequence
  source 1..14: mol_type = other DNA
tgctacaacttcct

SEQ ID NO: 635 - DNA, 15 bp, synthetic construct
  misc_feature 1..15: note = synthetic sequence
  source 1..15: mol_type = other DNA
tcgtgctacaacttc

SEQ ID NO: 636 - DNA, 14 bp, synthetic construct
  misc_feature 1..14: note = synthetic sequence
  source 1..14: mol_type = other DNA
cgtgctacaacttc

SEQ ID NO: 637 - DNA, 15 bp, synthetic construct
  misc_feature 1..15: note = synthetic sequence
  source 1..15: mol_type = other DNA
cctatatggaagagc

SEQ ID NO: 638 - DNA, 16 bp, synthetic construct
  misc_feature 1..16: note = synthetic sequence
  source 1..16: mol_type = other DNA
tgcctatatggaagag

SEQ ID NO: 639 - DNA, 15 bp, synthetic construct
  misc_feature 1..15: note = synthetic sequence
  source 1..15: mol_type = other DNA
gcctatatggaagag

SEQ ID NO: 640 - DNA, 14 bp, synthetic construct
  misc_feature 1..14: note = synthetic sequence
  source 1..14: mol_type = other DNA
tatatggaagagcc

SEQ ID NO: 641 - DNA, 16 bp, synthetic construct
  misc_feature 1..16: note = synthetic sequence
  source 1..16: mol_type = other DNA
agagccctaatgtgta

SEQ ID NO: 642 - DNA, 16 bp, synthetic construct
  misc_feature 1..16: note = synthetic sequence
  source 1..16: mol_type = other DNA
gaagagccctaatgtg

SEQ ID NO: 643 - DNA, 16 bp, synthetic construct
  misc_feature 1..16: note = synthetic sequence
  source 1..16: mol_type = other DNA
tgtgtaacattaggga

SEQ ID NO: 644 - DNA, 16 bp, synthetic construct
  misc_feature 1..16: note = synthetic sequence
  source 1..16: mol_type = other DNA
gtaacattagggagga

SEQ ID NO: 645 - DNA, 15 bp, synthetic construct
  misc_feature 1..15: note = synthetic sequence
  source 1..15: mol_type = other DNA
gtagtgttggtttta

SEQ ID NO: 646 - DNA, 14 bp, synthetic construct
  misc_feature 1..14: note = synthetic sequence
  source 1..14: mol_type = other DNA
gtagtgttggtttt

SEQ ID NO: 647 - DNA, 16 bp, synthetic construct
  misc_feature 1..16: note = synthetic sequence
  source 1..16: mol_type = other DNA
tcatgtggtagtgttg

SEQ ID NO: 648 - DNA, 15 bp, synthetic construct
  misc_feature 1..15: note = synthetic sequence
  source 1..15: mol_type = other DNA
tcatgtggtagtgtt

SEQ ID NO: 649 - DNA, 16 bp, synthetic construct
  misc_feature 1..16: note = synthetic sequence
  source 1..16: mol_type = other DNA
atgtggtagtgttggt

SEQ ID NO: 650 - DNA, 15 bp, synthetic construct
  misc_feature 1..15: note = synthetic sequence
  source 1..15: mol_type = other DNA
atgtggtagtgttgg

SEQ ID NO: 651 - DNA, 15 bp, synthetic construct
  misc_feature 1..15: note = synthetic sequence
  source 1..15: mol_type = other DNA
tgtggtagtgttggt

SEQ ID NO: 652 - DNA, 14 bp, synthetic construct
  misc_feature 1..14: note = synthetic sequence
  source 1..14: mol_type = other DNA
gtggtagtgttggt

SEQ ID NO: 653 - DNA, 16 bp, synthetic construct
  misc_feature 1..16: note = synthetic sequence
  source 1..16: mol_type = other DNA
gtggtagtgttggttt

SEQ ID NO: 654 - DNA, 15 bp, synthetic construct
  misc_feature 1..15: note = synthetic sequence
  source 1..15: mol_type = other DNA
tggtagtgttggttt

SEQ ID NO: 655 - DNA, 15 bp, synthetic construct
  misc_feature 1..15: note = synthetic sequence
  source 1..15: mol_type = other DNA
ggtttcgtccgtgtt

SEQ ID NO: 656 - DNA, 14 bp, synthetic construct
  misc_feature 1..14: note = synthetic sequence
  source 1..14: mol_type = other DNA
gtttcgtccgtgtt

SEQ ID NO: 657 - DNA, 15 bp, synthetic construct
  misc_feature 1..15: note = synthetic sequence
  source 1..15: mol_type = other DNA
gctgtcgcccgtgtc

SEQ ID NO: 658 - DNA, 15 bp, synthetic construct
  misc_feature 1..15: note = synthetic sequence
  source 1..15: mol_type = other DNA
gctgtcgcccgtgtc

SEQ ID NO: 659 - DNA, 15 bp, synthetic construct
  misc_feature 1..15: note = synthetic sequence
  source 1..15: mol_type = other DNA
gctgtcgcccgtgtc

SEQ ID NO: 660 - DNA, 14 bp, synthetic construct
  misc_feature 1..14: note = synthetic sequence
  source 1..14: mol_type = other DNA
gctgtcgcccgtgt

SEQ ID NO: 661 - DNA, 10 bp, synthetic construct
  misc_feature 1..10: note = synthetic sequence
  source 1..10: mol_type = other DNA
ttcgtccgtg

SEQ ID NO: 662 - DNA, 10 bp, synthetic construct
  misc_feature 1..10: note = synthetic sequence
  source 1..10: mol_type = other DNA
ttcgtccgtg

SEQ ID NO: 663 - DNA, 10 bp, synthetic construct
  misc_feature 1..10: note = synthetic sequence
  source 1..10: mol_type = other DNA
ttcgtccgtg

SEQ ID NO: 664-666 - skipped (3 entries)

SEQ ID NO: 667 - DNA, 10 bp, synthetic construct
  misc_feature 1..10: note = synthetic sequence
  source 1..10: mol_type = other DNA
tttcgtccgt

SEQ ID NO: 668 - DNA, 10 bp, synthetic construct
  misc_feature 1..10: note = synthetic sequence
  source 1..10: mol_type = other DNA
tttcgtccgt

SEQ ID NO: 669 - DNA, 10 bp, synthetic construct
  misc_feature 1..10: note = synthetic sequence
  source 1..10: mol_type = other DNA
tttcgtccgt

SEQ ID NO: 670 - DNA, 10 bp, synthetic construct
  misc_feature 1..10: note = synthetic sequence
  source 1..10: mol_type = other DNA
ccccacccac

SEQ ID NO: 671 - DNA, 10 bp, synthetic construct
  misc_feature 1..10: note = synthetic sequence
  source 1..10: mol_type = other DNA
ccccacccac

SEQ ID NO: 672 - DNA, 10 bp, synthetic construct
  misc_feature 1..10: note = synthetic sequence
  source 1..10: mol_type = other DNA
ccccacccac

SEQ ID NO: 673 - DNA, 12 bp, synthetic construct
  misc_feature 1..12: note = synthetic sequence
  source 1..12: mol_type = other DNA
tttcgtccgtgt

SEQ ID NO: 674 - DNA, 12 bp, synthetic construct
  misc_feature 1..12: note = synthetic sequence
  source 1..12: mol_type = other DNA
tttcgtccgtgt

SEQ ID NO: 675 - DNA, 12 bp, synthetic construct
  misc_feature 1..12: note = synthetic sequence
  source 1..12: mol_type = other DNA
tttcgtccgtgt

SEQ ID NO: 676 - DNA, 12 bp, synthetic construct
  misc_feature 1..12: note = synthetic sequence
  source 1..12: mol_type = other DNA
ttccatccatgt

SEQ ID NO: 677 - DNA, 12 bp, synthetic construct
  misc_feature 1..12: note = synthetic sequence
  source 1..12: mol_type = other DNA
ttccatccatgt

SEQ ID NO: 678 - DNA, 12 bp, synthetic construct
  misc_feature 1..12: note = synthetic sequence
  source 1..12: mol_type = other DNA
ttccatccatgt

SEQ ID NO: 679 - DNA, 12 bp, synthetic construct
  misc_feature 1..12: note = synthetic sequence
  source 1..12: mol_type = other DNA
ttccatccatgt

SEQ ID NO: 680 - DNA, 14 bp, synthetic construct
  misc_feature 1..14: note = synthetic sequence
  source 1..14: mol_type = other DNA
gtttcgtccgtgtt

SEQ ID NO: 681 - DNA, 14 bp, synthetic construct
  misc_feature 1..14: note = synthetic sequence
  source 1..14: mol_type = other DNA
gtttcgtccgtgtt

SEQ ID NO: 682 - DNA, 14 bp, synthetic construct
  misc_feature 1..14: note = synthetic sequence
  source 1..14: mol_type = other DNA
gtttcgtccgtgtt

SEQ ID NO: 683 - DNA, 14 bp, synthetic construct
  misc_feature 1..14: note = synthetic sequence
  source 1..14: mol_type = other DNA
gtttcggccatgtg

SEQ ID NO: 684 - DNA, 14 bp, synthetic construct
  misc_feature 1..14: note = synthetic sequence
  source 1..14: mol_type = other DNA
gtttcggccatgtg

SEQ ID NO: 685 - DNA, 14 bp, synthetic construct
  misc_feature 1..14: note = synthetic sequence
  source 1..14: mol_type = other DNA
gtttcggccatgtg

SEQ ID NO: 686 - DNA, 14 bp, synthetic construct
  misc_feature 1..14: note = synthetic sequence
  source 1..14: mol_type = other DNA
gtttcggccatgtg

SEQ ID NO: 687 - DNA, 10 bp, synthetic construct
  misc_feature 1..10: note = synthetic sequence
  source 1..10: mol_type = other DNA
cgtccgtgtt

SEQ ID NO: 688 - DNA, 10 bp, synthetic construct
  misc_feature 1..10: note = synthetic sequence
  source 1..10: mol_type = other DNA
cgtccgtgtt

SEQ ID NO: 689 - DNA, 10 bp, synthetic construct
  misc_feature 1..10: note = synthetic sequence
  source 1..10: mol_type = other DNA
cgtccgtgtt

SEQ ID NO: 690 - DNA, 10 bp, synthetic construct
  misc_feature 1..10: note = synthetic sequence
  source 1..10: mol_type = other DNA
cgtccgtgtt

SEQ ID NO: 691 - DNA, 10 bp, synthetic construct
  misc_feature 1..10: note = synthetic sequence
  source 1..10: mol_type = other DNA
cctccgtgtc

SEQ ID NO: 692 - DNA, 10 bp, synthetic construct
  misc_feature 1..10: note = synthetic sequence
  source 1..10: mol_type = other DNA
cctccgtgtc

SEQ ID NO: 693 - DNA, 10 bp, synthetic construct
  misc_feature 1..10: note = synthetic sequence
  source 1..10: mol_type = other DNA
cctccgtgtc

SEQ ID NO: 694 - DNA, 10 bp, synthetic construct
  misc_feature 1..10: note = synthetic sequence
  source 1..10: mol_type = other DNA
tccgtgttgc

SEQ ID NO: 695 - DNA, 10 bp, synthetic construct
  misc_feature 1..10: note = synthetic sequence
  source 1..10: mol_type = other DNA
tccgtgttgc

SEQ ID NO: 696 - DNA, 10 bp, synthetic construct
  misc_feature 1..10: note = synthetic sequence
  source 1..10: mol_type = other DNA
tccgtgttgc

SEQ ID NO: 697 - DNA, 10 bp, synthetic construct
  misc_feature 1..10: note = synthetic sequence
  source 1..10: mol_type = other DNA
tccgtcttgc

SEQ ID NO: 698 - DNA, 10 bp, synthetic construct
  misc_feature 1..10: note = synthetic sequence
  source 1..10: mol_type = other DNA
tccgtcttgc

SEQ ID NO: 699 - skipped

SEQ ID NO: 700 - DNA, 13 bp, synthetic construct
  misc_feature 1..13: note = synthetic sequence
  source 1..13: mol_type = other DNA
tttcgtccgtgtt

SEQ ID NO: 701 - DNA, 13 bp, synthetic construct
  misc_feature 1..13: note = synthetic sequence
  source 1..13: mol_type = other DNA
tttcgtccgtgtt

SEQ ID NO: 702 - DNA, 13 bp, synthetic construct
  misc_feature 1..13: note = synthetic sequence
  source 1..13: mol_type = other DNA
tttcctctatgtt

SEQ ID NO: 703 - DNA, 13 bp, synthetic construct
  misc_feature 1..13: note = synthetic sequence
  source 1..13: mol_type = other DNA
tttcctctatgtt

SEQ ID NO: 704 - DNA, 13 bp, synthetic construct
  misc_feature 1..13: note = synthetic sequence
  source 1..13: mol_type = other DNA
gtttcgtccgtgt

SEQ ID NO: 705 - DNA, 15 bp, synthetic construct
  misc_feature 1..15: note = synthetic sequence
  source 1..15: mol_type = other DNA
ggtttcgtccgtgtt

SEQ ID NO: 706 - DNA, 15 bp, synthetic construct
  misc_feature 1..15: note = synthetic sequence
  source 1..15: mol_type = other DNA
ggtttcgtccgtgtt

SEQ ID NO: 707 - DNA, 15 bp, synthetic construct
  misc_feature 1..15: note = synthetic sequence
  source 1..15: mol_type = other DNA
ggtttcgtccgtgtt

SEQ ID NO: 708 - DNA, 15 bp, synthetic construct
  misc_feature 1..15: note = synthetic sequence
  source 1..15: mol_type = other DNA
aagtacgtcctactt

SEQ ID NO: 709 - DNA, 10 bp, synthetic construct
  misc_feature 1..10: note = synthetic sequence
  source 1..10: mol_type = other DNA
ggtttcgtcc

SEQ ID NO: 710 - DNA, 10 bp, synthetic construct
  misc_feature 1..10: note = synthetic sequence
  source 1..10: mol_type = other DNA
ggtttcgtcc

SEQ ID NO: 711 - DNA, 15 bp, synthetic construct
  misc_feature 1..15: note = synthetic sequence
  source 1..15: mol_type = other DNA
tgggtttcgtccgtt

SEQ ID NO: 712 - DNA, 14 bp, synthetic construct
  misc_feature 1..14: note = synthetic sequence
  source 1..14: mol_type = other DNA
ttttgggattccgt

SEQ ID NO: 713 - DNA, 16 bp, synthetic construct
  misc_feature 1..16: note = synthetic sequence
  source 1..16: mol_type = other DNA
gcttttgggattccgt

SEQ ID NO: 714 - DNA, 16 bp, synthetic construct
  misc_feature 1..16: note = synthetic sequence
  source 1..16: mol_type = other DNA
gcttttgggattccgt

SEQ ID NO: 715 - DNA, 16 bp, synthetic construct
  misc_feature 1..16: note = synthetic sequence
  source 1..16: mol_type = other DNA
agctgcttttgggatt

SEQ ID NO: 716 - DNA, 16 bp, synthetic construct
  misc_feature 1..16: note = synthetic sequence
  source 1..16: mol_type = other DNA
gagctgcttttgggat

SEQ ID NO: 717 - DNA, 16 bp, synthetic construct
  misc_feature 1..16: note = synthetic sequence
  source 1..16: mol_type = other DNA
ctgcttttgggattcc

SEQ ID NO: 718 - DNA, 14 bp, synthetic construct
  misc_feature 1..14: note = synthetic sequence
  source 1..14: mol_type = other DNA
tgcttttgggattc

SEQ ID NO: 719 - DNA, 14 bp, synthetic construct
  misc_feature 1..14: note = synthetic sequence
  source 1..14: mol_type = other DNA
tgcttttgggattc

SEQ ID NO: 720 - DNA, 16 bp, synthetic construct
  misc_feature 1..16: note = synthetic sequence
  source 1..16: mol_type = other DNA
agctgcttttgggatt

SEQ ID NO: 721 - DNA, 14 bp, synthetic construct
  misc_feature 1..14: note = synthetic sequence
  source 1..14: mol_type = other DNA
agctgcttttggga

SEQ ID NO: 722 - DNA, 16 bp, synthetic construct
  misc_feature 1..16: note = synthetic sequence
  source 1..16: mol_type = other DNA
cagctgcttttgggat

SEQ ID NO: 723 - DNA, 16 bp, synthetic construct
  misc_feature 1..16: note = synthetic sequence
  source 1..16: mol_type = other DNA
agctgcttttgggatt

SEQ ID NO: 724 - DNA, 14 bp, synthetic construct
  misc_feature 1..14: note = synthetic sequence
  source 1..14: mol_type = other DNA
agctgcttttggga

SEQ ID NO: 725 - DNA, 14 bp, synthetic construct
  misc_feature 1..14: note = synthetic sequence
  source 1..14: mol_type = other DNA
agctgcttttggga

SEQ ID NO: 726 - DNA, 16 bp, synthetic construct
  misc_feature 1..16: note = synthetic sequence
  source 1..16: mol_type = other DNA
agctgcttttgggatt

SEQ ID NO: 727 - DNA, 14 bp, synthetic construct
  misc_feature 1..14: note = synthetic sequence
  source 1..14: mol_type = other DNA
tgcttttgggattc

SEQ ID NO: 728 - DNA, 14 bp, synthetic construct
  misc_feature 1..14: note = synthetic sequence
  source 1..14: mol_type = other DNA
gcggcgccccgcct

SEQ ID NO: 729 - DNA, 14 bp, synthetic construct
  misc_feature 1..14: note = synthetic sequence
  source 1..14: mol_type = other DNA
gcggcgccccgcct

SEQ ID NO: 730 - DNA, 21 bp, synthetic construct
  misc_feature 1..21: note = synthetic sequence
  source 1..21: mol_type = other DNA
cggtcccgcggcgccccgcct

SEQ ID NO: 731 - DNA, 16 bp, synthetic construct
  misc_feature 1..16: note = synthetic sequence
  source 1..16: mol_type = other DNA
tttgggcttcctcgct

SEQ ID NO: 732 - DNA, 16 bp, synthetic construct
  misc_feature 1..16: note = synthetic sequence
  source 1..16: mol_type = other DNA
tttgggcttcctcgct

SEQ ID NO: 733 - DNA, 14 bp, synthetic construct
  misc_feature 1..14: note = synthetic sequence
  source 1..14: mol_type = other DNA
tttgggcttcctcg

SEQ ID NO: 734 - DNA, 14 bp, synthetic construct
  misc_feature 1..14: note = synthetic sequence
  source 1..14: mol_type = other DNA
tttgggcttcctcg

SEQ ID NO: 735 - DNA, 14 bp, synthetic construct
  misc_feature 1..14: note = synthetic sequence
  source 1..14: mol_type = other DNA
tgggcttcctcgct

SEQ ID NO: 736 - DNA, 16 bp, synthetic construct
  misc_feature 1..16: note = synthetic sequence
  source 1..16: mol_type = other DNA
atatactttgggcttc

SEQ ID NO: 737 - DNA, 16 bp, synthetic construct
  misc_feature 1..16: note = synthetic sequence
  source 1..16: mol_type = other DNA
atatactttgggcttc

SEQ ID NO: 738 - DNA, 14 bp, synthetic construct
  misc_feature 1..14: note = synthetic sequence
  source 1..14: mol_type = other DNA
atatactttgggct

SEQ ID NO: 739 - DNA, 15 bp, synthetic construct
  misc_feature 1..15: note = synthetic sequence
  source 1..15: mol_type = other DNA
atatactttgggctt

SEQ ID NO: 740 - DNA, 16 bp, synthetic construct
  misc_feature 1..16: note = synthetic sequence
  source 1..16: mol_type = other DNA
tagccctagccccgca

SEQ ID NO: 741 - DNA, 16 bp, synthetic construct
  misc_feature 1..16: note = synthetic sequence
  source 1..16: mol_type = other DNA
tagccctagccccgca

SEQ ID NO: 742 - DNA, 14 bp, synthetic construct
  misc_feature 1..14: note = synthetic sequence
  source 1..14: mol_type = other DNA
tagccctagccccg

SEQ ID NO: 743 - DNA, 14 bp, synthetic construct
  misc_feature 1..14: note = synthetic sequence
  source 1..14: mol_type = other DNA
tgctgttagcccta

SEQ ID NO: 744 - DNA, 14 bp, synthetic construct
  misc_feature 1..14: note = synthetic sequence
  source 1..14: mol_type = other DNA
tgctgttagcccta

SEQ ID NO: 745 - DNA, 14 bp, synthetic construct
  misc_feature 1..14: note = synthetic sequence
  source 1..14: mol_type = other DNA
tgctgttagcccta

SEQ ID NO: 746 - DNA, 15 bp, synthetic construct
  misc_feature 1..15: note = synthetic sequence
  source 1..15: mol_type = other DNA
gtgttagccctagcc

SEQ ID NO: 747 - DNA, 14 bp, synthetic construct
  misc_feature 1..14: note = synthetic sequence
  source 1..14: mol_type = other DNA
gcgcccagccccgc

SEQ ID NO: 748 - DNA, 14 bp, synthetic construct
  misc_feature 1..14: note = synthetic sequence
  source 1..14: mol_type = other DNA
gcgcccagccccgc

SEQ ID NO: 749 - DNA, 14 bp, synthetic construct
  misc_feature 1..14: note = synthetic sequence
  source 1..14: mol_type = other DNA
cgcgcgcccagccc

SEQ ID NO: 750 - DNA, 17 bp, synthetic construct
  misc_feature 1..17: note = synthetic sequence
  source 1..17: mol_type = other DNA
cgcgcgcccagccccgc

SEQ ID NO: 751 - DNA, 16 bp, synthetic construct
  misc_feature 1..16: note = synthetic sequence
  source 1..16: mol_type = other DNA
tggcatggaatgggct

SEQ ID NO: 752 - DNA, 14 bp, synthetic construct
  misc_feature 1..14: note = synthetic sequence
  source 1..14: mol_type = other DNA
tggcatggaatggg

SEQ ID NO: 753 - DNA, 16 bp, synthetic construct
  misc_feature 1..16: note = synthetic sequence
  source 1..16: mol_type = other DNA
atggaatgggctccgc

SEQ ID NO: 754 - DNA, 14 bp, synthetic construct
  misc_feature 1..14: note = synthetic sequence
  source 1..14: mol_type = other DNA
atggaatgggctcc

SEQ ID NO: 755 - DNA, 15 bp, synthetic construct
  misc_feature 1..15: note = synthetic sequence
  source 1..15: mol_type = other DNA
aatgggctccgccag

SEQ ID NO: 756 - DNA, 15 bp, synthetic construct
  misc_feature 1..15: note = synthetic sequence
  source 1..15: mol_type = other DNA
aatgggctccgccag

SEQ ID NO: 757 - DNA, 14 bp, synthetic construct
  misc_feature 1..14: note = synthetic sequence
  source 1..14: mol_type = other DNA
aatgggctccgcca

SEQ ID NO: 758 - DNA, 14 bp, synthetic construct
  misc_feature 1..14: note = synthetic sequence
  source 1..14: mol_type = other DNA
aatgggctccgcca

SEQ ID NO: 759 - DNA, 16 bp, synthetic construct
  misc_feature 1..16: note = synthetic sequence
  source 1..16: mol_type = other DNA
cttacccgaggcggtc

SEQ ID NO: 760 - DNA, 14 bp, synthetic construct
  misc_feature 1..14: note = synthetic sequence
  source 1..14: mol_type = other DNA
ttacccgaggcggt

SEQ ID NO: 761 - DNA, 16 bp, synthetic construct
  misc_feature 1..16: note = synthetic sequence
  source 1..16: mol_type = other DNA
accgtaccttacccga

SEQ ID NO: 762 - DNA, 14 bp, synthetic construct
  misc_feature 1..14: note = synthetic sequence
  source 1..14: mol_type = other DNA
cgtaccttacccga

SEQ ID NO: 763 - DNA, 14 bp, synthetic construct
  misc_feature 1..14: note = synthetic sequence
  source 1..14: mol_type = other DNA
cgtaccttacccga

SEQ ID NO: 764 - DNA, 14 bp, synthetic construct
  misc_feature 1..14: note = synthetic sequence
  source 1..14: mol_type = other DNA
ctccgagccccgcc

SEQ ID NO: 765 - DNA, 19 bp, synthetic construct
  misc_feature 1..19: note = synthetic sequence
  source 1..19: mol_type = other DNA
cccggctccgagccccgcc

SEQ ID NO: 766 - DNA, 15 bp, synthetic construct
  misc_feature 1..15: note = synthetic sequence
  source 1..15: mol_type = other DNA
tggcctgtccccgca

SEQ ID NO: 767 - DNA, 15 bp, synthetic construct
  misc_feature 1..15: note = synthetic sequence
  source 1..15: mol_type = other DNA
tggcctgtccccgca

SEQ ID NO: 768 - DNA, 14 bp, synthetic construct
  misc_feature 1..14: note = synthetic sequence
  source 1..14: mol_type = other DNA
gatgccctggcctg

SEQ ID NO: 769 - DNA, 14 bp, synthetic construct
  misc_feature 1..14: note = synthetic sequence
  source 1..14: mol_type = other DNA
gatgccctggcctg

SEQ ID NO: 770 - DNA, 14 bp, synthetic construct
  misc_feature 1..14: note = synthetic sequence
  source 1..14: mol_type = other DNA
gcagccagctctac

SEQ ID NO: 771 - DNA, 14 bp, synthetic construct
  misc_feature 1..14: note = synthetic sequence
  source 1..14: mol_type = other DNA
gcagccagctctac

SEQ ID NO: 772 - DNA, 14 bp, synthetic construct
  misc_feature 1..14: note = synthetic sequence
  source 1..14: mol_type = other DNA
agccagctctaccc

SEQ ID NO: 773 - DNA, 16 bp, synthetic construct
  misc_feature 1..16: note = synthetic sequence
  source 1..16: mol_type = other DNA
agctctacccccgcca

SEQ ID NO: 774 - DNA, 16 bp, synthetic construct
  misc_feature 1..16: note = synthetic sequence
  source 1..16: mol_type = other DNA
agctctacccccgcca

SEQ ID NO: 775 - DNA, 16 bp, synthetic construct
  misc_feature 1..16: note = synthetic sequence
  source 1..16: mol_type = other DNA
aaagcagcgcccactt

SEQ ID NO: 776 - DNA, 15 bp, synthetic construct
  misc_feature 1..15: note = synthetic sequence
  source 1..15: mol_type = other DNA
aaagcagcgcccact

SEQ ID NO: 777 - DNA, 14 bp, synthetic construct
  misc_feature 1..14: note = synthetic sequence
  source 1..14: mol_type = other DNA
aaagcagcgcccac

SEQ ID NO: 778 - DNA, 14 bp, synthetic construct
  misc_feature 1..14: note = synthetic sequence
  source 1..14: mol_type = other DNA
acttcctccccgct

SEQ ID NO: 779 - DNA, 16 bp, synthetic construct
  misc_feature 1..16: note = synthetic sequence
  source 1..16: mol_type = other DNA
ctacagaagccccata

SEQ ID NO: 780 - DNA, 16 bp, synthetic construct
  misc_feature 1..16: note = synthetic sequence
  source 1..16: mol_type = other DNA
ctacagaagccccata

SEQ ID NO: 781 - DNA, 16 bp, synthetic construct
  misc_feature 1..16: note = synthetic sequence
  source 1..16: mol_type = other DNA
gaaatctctacagaag

SEQ ID NO: 782 - DNA, 16 bp, synthetic construct
  misc_feature 1..16: note = synthetic sequence
  source 1..16: mol_type = other DNA
gaaatctctacagaag

SEQ ID NO: 783 - DNA, 16 bp, synthetic construct
  misc_feature 1..16: note = synthetic sequence
  source 1..16: mol_type = other DNA
tgatccctgtccccat

SEQ ID NO: 784 - DNA, 15 bp, synthetic construct
  misc_feature 1..15: note = synthetic sequence
  source 1..15: mol_type = other DNA
atgctgatccctgtc

SEQ ID NO: 785 - DNA, 23 bp, synthetic construct
  misc_feature 1..23: note = synthetic sequence
  source 1..23: mol_type = other DNA
gccatgctgatccctgtccccat

SEQ ID NO: 786 - DNA, 14 bp, synthetic construct
  misc_feature 1..14: note = synthetic sequence
  source 1..14: mol_type = other DNA
ccatctcaccccat

SEQ ID NO: 787 - DNA, 15 bp, synthetic construct
  misc_feature 1..15: note = synthetic sequence
  source 1..15: mol_type = other DNA
gctgctcctccccat

SEQ ID NO: 788 - DNA, 15 bp, synthetic construct
  misc_feature 1..15: note = synthetic sequence
  source 1..15: mol_type = other DNA
tctccaaccccacaa

SEQ ID NO: 789 - DNA, 14 bp, synthetic construct
  misc_feature 1..14: note = synthetic sequence
  source 1..14: mol_type = other DNA
ctccaaccccacaa

SEQ ID NO: 790 - DNA, 15 bp, synthetic construct
  misc_feature 1..15: note = synthetic sequence
  source 1..15: mol_type = other DNA
cagccagctctccaa

SEQ ID NO: 791 - DNA, 14 bp, synthetic construct
  misc_feature 1..14: note = synthetic sequence
  source 1..14: mol_type = other DNA
agccagctctccaa

SEQ ID NO: 792 - DNA, 16 bp, synthetic construct
  misc_feature 1..16: note = synthetic sequence
  source 1..16: mol_type = other DNA
gacgtgatatatgtgg

SEQ ID NO: 793 - DNA, 16 bp, synthetic construct
  misc_feature 1..16: note = synthetic sequence
  source 1..16: mol_type = other DNA
cgtgatatatgtggta

SEQ ID NO: 794 - DNA, 15 bp, synthetic construct
  misc_feature 1..15: note = synthetic sequence
  source 1..15: mol_type = other DNA
gatatgtggtaccat

SEQ ID NO: 795 - DNA, 14 bp, synthetic construct
  misc_feature 1..14: note = synthetic sequence
  source 1..14: mol_type = other DNA
tggtaccatgtcac

SEQ ID NO: 796 - DNA, 16 bp, synthetic construct
  misc_feature 1..16: note = synthetic sequence
  source 1..16: mol_type = other DNA
cctcagcagcagattt

SEQ ID NO: 797 - DNA, 15 bp, synthetic construct
  misc_feature 1..15: note = synthetic sequence
  source 1..15: mol_type = other DNA
tcagcagcagatttc

SEQ ID NO: 798 - DNA, 14 bp, synthetic construct
  misc_feature 1..14: note = synthetic sequence
  source 1..14: mol_type = other DNA
cagcagcagatttc

SEQ ID NO: 799 - DNA, 16 bp, synthetic construct
  misc_feature 1..16: note = synthetic sequence
  source 1..16: mol_type = other DNA
cagatttcttagtgac

SEQ ID NO: 800 - DNA, 16 bp, synthetic construct
  misc_feature 1..16: note = synthetic sequence
  source 1..16: mol_type = other DNA
tgcaacacggacgaaa

SEQ ID NO: 801 - DNA, 16 bp, synthetic construct
  misc_feature 1..16: note = synthetic sequence
  source 1..16: mol_type = other DNA
gcaacacggacgaaac

SEQ ID NO: 802 - DNA, 15 bp, synthetic construct
  misc_feature 1..15: note = synthetic sequence
  source 1..15: mol_type = other DNA
acacggacgaaaccg

SEQ ID NO: 803 - DNA, 15 bp, synthetic construct
  misc_feature 1..15: note = synthetic sequence
  source 1..15: mol_type = other DNA
ggacgaaacccgtaa

SEQ ID NO: 804 - DNA, 15 bp, synthetic construct
  misc_feature 1..15: note = synthetic sequence
  source 1..15: mol_type = other DNA
acgaaaccgtaagca

SEQ ID NO: 805 - DNA, 15 bp, synthetic construct
  misc_feature 1..15: note = synthetic sequence
  source 1..15: mol_type = other DNA
acgaaaccgtaagca

SEQ ID NO: 806 - DNA, 16 bp, synthetic construct
  misc_feature 1..16: note = synthetic sequence
  source 1..16: mol_type = other DNA
gcaacacggacgaaac

SEQ ID NO: 807 - DNA, 15 bp, synthetic construct
  misc_feature 1..15: note = synthetic sequence
  source 1..15: mol_type = other DNA
gcaacacggacgaaa

SEQ ID NO: 808 - DNA, 16 bp, synthetic construct
  misc_feature 1..16: note = synthetic sequence
  source 1..16: mol_type = other DNA
gcaacacggacgaaac

SEQ ID NO: 809 - DNA, 16 bp, synthetic construct
  misc_feature 1..16: note = synthetic sequence
  source 1..16: mol_type = other DNA
gcaacacggacgaaac

SEQ ID NO: 810 - DNA, 16 bp, synthetic construct
  misc_feature 1..16: note = synthetic sequence
  source 1..16: mol_type = other DNA
gcaacacggacgaaac

SEQ ID NO: 811 - DNA, 14 bp, synthetic construct
  misc_feature 1..14: note = synthetic sequence
  source 1..14: mol_type = other DNA
gcaacacggacgaa

SEQ ID NO: 812 - DNA, 15 bp, synthetic construct
  misc_feature 1..15: note = synthetic sequence
  source 1..15: mol_type = other DNA
acacggacgaaaccg

SEQ ID NO: 813 - DNA, 15 bp, synthetic construct
  misc_feature 1..15: note = synthetic sequence
  source 1..15: mol_type = other DNA
acacggacgaaaccg

SEQ ID NO: 814 - DNA, 16 bp, synthetic construct
  misc_feature 1..16: note = synthetic sequence
  source 1..16: mol_type = other DNA
aacacggacgaaaccg

SEQ ID NO: 815 - DNA, 16 bp, synthetic construct
  misc_feature 1..16: note = synthetic sequence
  source 1..16: mol_type = other DNA
aacacggacgaaaccg

SEQ ID NO: 816 - DNA, 15 bp, synthetic construct
  misc_feature 1..15: note = synthetic sequence
  source 1..15: mol_type = other DNA
acgaaaccgtaagca

SEQ ID NO: 817 - DNA, 15 bp, synthetic construct
  misc_feature 1..15: note = synthetic sequence
  source 1..15: mol_type = other DNA
acgaaaccgtaagca

SEQ ID NO: 818 - DNA, 16 bp, synthetic construct
  misc_feature 1..16: note = synthetic sequence
  source 1..16: mol_type = other DNA
aacatgtctggaccta

SEQ ID NO: 819 - DNA, 16 bp, synthetic construct
  misc_feature 1..16: note = synthetic sequence
  source 1..16: mol_type = other DNA
acatgtctggacctat

SEQ ID NO: 820 - DNA, 15 bp, synthetic construct
  misc_feature 1..15: note = synthetic sequence
  source 1..15: mol_type = other DNA
tgaatatgacatagt

SEQ ID NO: 821 - DNA, 14 bp, synthetic construct
  misc_feature 1..14: note = synthetic sequence
  source 1..14: mol_type = other DNA
aatatgacatagtc

SEQ ID NO: 822 - DNA, 16 bp, synthetic construct
  misc_feature 1..16: note = synthetic sequence
  source 1..16: mol_type = other DNA
cacagattttaaagtt

SEQ ID NO: 823 - DNA, 16 bp, synthetic construct
  misc_feature 1..16: note = synthetic sequence
  source 1..16: mol_type = other DNA
cacagattttaaagtt

SEQ ID NO: 824 - DNA, 16 bp, synthetic construct
  misc_feature 1..16: note = synthetic sequence
  source 1..16: mol_type = other DNA
cagattttaaagttcg

SEQ ID NO: 825 - DNA, 15 bp, synthetic construct
  misc_feature 1..15: note = synthetic sequence
  source 1..15: mol_type = other DNA
gattttaaagttcgt

SEQ ID NO: 826 - DNA, 15 bp, synthetic construct
  misc_feature 1..15: note = synthetic sequence
  source 1..15: mol_type = other DNA
taaagttcgtttaga

SEQ ID NO: 827 - DNA, 14 bp, synthetic construct
  misc_feature 1..14: note = synthetic sequence
  source 1..14: mol_type = other DNA
aaagttcgtttaga

SEQ ID NO: 828 - DNA, 17 bp, synthetic construct
  misc_feature 1..17: note = synthetic sequence
  source 1..17: mol_type = other DNA
tcgtttagagaacagat

SEQ ID NO: 829 - DNA, 16 bp, synthetic construct
  misc_feature 1..16: note = synthetic sequence
  source 1..16: mol_type = other DNA
agagaacagatctaca

SEQ ID NO: 830 - DNA, 14 bp, synthetic construct
  misc_feature 1..14: note = synthetic sequence
  source 1..14: mol_type = other DNA
agatctacaagaga

SEQ ID NO: 831 - DNA, 14 bp, synthetic construct
  misc_feature 1..14: note = synthetic sequence
  source 1..14: mol_type = other DNA
atctacaagagatc

SEQ ID NO: 832 - DNA, 16 bp, synthetic construct
  misc_feature 1..16: note = synthetic sequence
  source 1..16: mol_type = other DNA
agattttaaagttcgt

SEQ ID NO: 833 - DNA, 15 bp, synthetic construct
  misc_feature 1..15: note = synthetic sequence
  source 1..15: mol_type = other DNA
gattttaaagttcgt

SEQ ID NO: 834 - DNA, 15 bp, synthetic construct
  misc_feature 1..15: note = synthetic sequence
  source 1..15: mol_type = other DNA
gattttaaagttcgt

SEQ ID NO: 835 - DNA, 15 bp, synthetic construct
  misc_feature 1..15: note = synthetic sequence
  source 1..15: mol_type = other DNA
agattttaaagttcg

SEQ ID NO: 836 - DNA, 17 bp, synthetic construct
  misc_feature 1..17: note = synthetic sequence
  source 1..17: mol_type = other DNA
tcgtttagagaacagat

SEQ ID NO: 837 - DNA, 16 bp, synthetic construct
  misc_feature 1..16: note = synthetic sequence
  source 1..16: mol_type = other DNA
ttcgtttagagaacag

SEQ ID NO: 838 - DNA, 16 bp, synthetic construct
  misc_feature 1..16: note = synthetic sequence
  source 1..16: mol_type = other DNA
ttcgtttagagaacag

SEQ ID NO: 839 - DNA, 16 bp, synthetic construct
  misc_feature 1..16: note = synthetic sequence
  source 1..16: mol_type = other DNA
caggcaaactgagttg

SEQ ID NO: 840 - DNA, 16 bp, synthetic construct
  misc_feature 1..16: note = synthetic sequence
  source 1..16: mol_type = other DNA
caggcaaactgagttg

SEQ ID NO: 841 - DNA, 14 bp, synthetic construct
  misc_feature 1..14: note = synthetic sequence
  source 1..14: mol_type = other DNA
caggcaaactgagt

SEQ ID NO: 842 - DNA, 16 bp, synthetic construct
  misc_feature 1..16: note = synthetic sequence
  source 1..16: mol_type = other DNA
caaactgagttggacg

SEQ ID NO: 843 - DNA, 14 bp, synthetic construct
  misc_feature 1..14: note = synthetic sequence
  source 1..14: mol_type = other DNA
aaactgagttggac

SEQ ID NO: 844 - DNA, 16 bp, synthetic construct
  misc_feature 1..16: note = synthetic sequence
  source 1..16: mol_type = other DNA
aaactgagttggacgt

SEQ ID NO: 845 - DNA, 15 bp, synthetic construct
  misc_feature 1..15: note = synthetic sequence
  source 1..15: mol_type = other DNA
gagttggacgtgtgt

SEQ ID NO: 846 - DNA, 16 bp, synthetic construct
  misc_feature 1..16: note = synthetic sequence
  source 1..16: mol_type = other DNA
ttggacgtgtgttttc

SEQ ID NO: 847 - DNA, 16 bp, synthetic construct
  misc_feature 1..16: note = synthetic sequence
  source 1..16: mol_type = other DNA
ggacgtgtgttttctc

SEQ ID NO: 848 - DNA, 16 bp, synthetic construct
  misc_feature 1..16: note = synthetic sequence
  source 1..16: mol_type = other DNA
tttcggtcacacccgg

SEQ ID NO: 849 - DNA, 16 bp, synthetic construct
  misc_feature 1..16: note = synthetic sequence
  source 1..16: mol_type = other DNA
cggtcacacccggacg

SEQ ID NO: 850 - DNA, 16 bp, synthetic construct
  misc_feature 1..16: note = synthetic sequence
  source 1..16: mol_type = other DNA
tcacacccggacgaaa

SEQ ID NO: 851 - DNA, 14 bp, synthetic construct
  misc_feature 1..14: note = synthetic sequence
  source 1..14: mol_type = other DNA
cacccggacgaaac

SEQ ID NO: 852 - DNA, 15 bp, synthetic construct
  misc_feature 1..15: note = synthetic sequence
  source 1..15: mol_type = other DNA
cacccggacgaaacc

SEQ ID NO: 853 - DNA, 16 bp, synthetic construct
  misc_feature 1..16: note = synthetic sequence
  source 1..16: mol_type = other DNA
cacccggacgaaacct

SEQ ID NO: 854 - DNA, 14 bp, synthetic construct
  misc_feature 1..14: note = synthetic sequence
  source 1..14: mol_type = other DNA
ccggacgaaaccta

SEQ ID NO: 855 - DNA, 17 bp, synthetic construct
  misc_feature 1..17: note = synthetic sequence
  source 1..17: mol_type = other DNA
cggtcacacccggacga

SEQ ID NO: 856 - DNA, 16 bp, synthetic construct
  misc_feature 1..16: note = synthetic sequence
  source 1..16: mol_type = other DNA
cggtcacacccggacg

SEQ ID NO: 857 - DNA, 16 bp, synthetic construct
  misc_feature 1..16: note = synthetic sequence
  source 1..16: mol_type = other DNA
cggtcacacccggacg

SEQ ID NO: 858 - DNA, 16 bp, synthetic construct
  misc_feature 1..16: note = synthetic sequence
  source 1..16: mol_type = other DNA
cggtcacacccggacg

SEQ ID NO: 859 - DNA, 14 bp, synthetic construct
  misc_feature 1..14: note = synthetic sequence
  source 1..14: mol_type = other DNA
gtcacacccggacg

SEQ ID NO: 860 - DNA, 14 bp, synthetic construct
  misc_feature 1..14: note = synthetic sequence
  source 1..14: mol_type = other DNA
gtcacacccggacg

SEQ ID NO: 861 - DNA, 15 bp, synthetic construct
  misc_feature 1..15: note = synthetic sequence
  source 1..15: mol_type = other DNA
cacccggacgaaacc

SEQ ID NO: 862 - DNA, 15 bp, synthetic construct
  misc_feature 1..15: note = synthetic sequence
  source 1..15: mol_type = other DNA
cacccggacgaaacc

SEQ ID NO: 863 - DNA, 14 bp, synthetic construct
  misc_feature 1..14: note = synthetic sequence
  source 1..14: mol_type = other DNA
cacccggacgaaac

SEQ ID NO: 864 - DNA, 16 bp, synthetic construct
  misc_feature 1..16: note = synthetic sequence
  source 1..16: mol_type = other DNA
cacacccggacgaaac

SEQ ID NO: 865 - DNA, 15 bp, synthetic construct
  misc_feature 1..15: note = synthetic sequence
  source 1..15: mol_type = other DNA
cacacccggacgaaa

SEQ ID NO: 866 - DNA, 14 bp, synthetic construct
  misc_feature 1..14: note = synthetic sequence
  source 1..14: mol_type = other DNA
cacacccggacgaa

SEQ ID NO: 867 - DNA, 15 bp, synthetic construct
  misc_feature 1..15: note = synthetic sequence
  source 1..15: mol_type = other DNA
tcgatcgtactccgc

SEQ ID NO: 868 - DNA, 14 bp, synthetic construct
  misc_feature 1..14: note = synthetic sequence
  source 1..14: mol_type = other DNA
tcgatcgtactccg

SEQ ID NO: 869 - DNA, 15 bp, synthetic construct
  misc_feature 1..15: note = synthetic sequence
  source 1..15: mol_type = other DNA
atcgtactccgcgtg

SEQ ID NO: 870 - DNA, 14 bp, synthetic construct
  misc_feature 1..14: note = synthetic sequence
  source 1..14: mol_type = other DNA
actcgatcgtactc

SEQ ID NO: 871 - DNA, 15 bp, synthetic construct
  misc_feature 1..15: note = synthetic sequence
  source 1..15: mol_type = other DNA
cgtggcctcggtgaa

SEQ ID NO: 872 - DNA, 14 bp, synthetic construct
  misc_feature 1..14: note = synthetic sequence
  source 1..14: mol_type = other DNA
gtggcctcggtgaa

SEQ ID NO: 873 - DNA, 16 bp, synthetic construct
  misc_feature 1..16: note = synthetic sequence
  source 1..16: mol_type = other DNA
gattaaagattgctat

SEQ ID NO: 874 - DNA, 16 bp, synthetic construct
  misc_feature 1..16: note = synthetic sequence
  source 1..16: mol_type = other DNA
taaagattgctatgtg

SEQ ID NO: 875 - DNA, 16 bp, synthetic construct
  misc_feature 1..16: note = synthetic sequence
  source 1..16: mol_type = other DNA
aagattgctatgtgag

SEQ ID NO: 876 - DNA, 16 bp, synthetic construct
  misc_feature 1..16: note = synthetic sequence
  source 1..16: mol_type = other DNA
gctatgtgagttaaag

SEQ ID NO: 877 - DNA, 16 bp, synthetic construct
  misc_feature 1..16: note = synthetic sequence
  source 1..16: mol_type = other DNA
tatgtgagttaaagtt

SEQ ID NO: 878 - DNA, 16 bp, synthetic construct
  misc_feature 1..16: note = synthetic sequence
  source 1..16: mol_type = other DNA
tgtgagttaaagttaa

SEQ ID NO: 879 - DNA, 16 bp, synthetic construct
  misc_feature 1..16: note = synthetic sequence
  source 1..16: mol_type = other DNA
tcgtagaagccttttg

SEQ ID NO: 880 - DNA, 17 bp, synthetic construct
  misc_feature 1..17: note = synthetic sequence
  source 1..17: mol_type = other DNA
cgtagaagccttttggc

SEQ ID NO: 881 - DNA, 16 bp, synthetic construct
  misc_feature 1..16: note = synthetic sequence
  source 1..16: mol_type = other DNA
tagaagccttttggca

SEQ ID NO: 882 - DNA, 16 bp, synthetic construct
  misc_feature 1..16: note = synthetic sequence
  source 1..16: mol_type = other DNA
aagccttttggcaatg

SEQ ID NO: 883 - DNA, 16 bp, synthetic construct
  misc_feature 1..16: note = synthetic sequence
  source 1..16: mol_type = other DNA
ttggcaatgttgttcc

SEQ ID NO: 884 - DNA, 14 bp, synthetic construct
  misc_feature 1..14: note = synthetic sequence
  source 1..14: mol_type = other DNA
gcaatgttgttcct

SEQ ID NO: 885 - DNA, 14 bp, synthetic construct
  misc_feature 1..14: note = synthetic sequence
  source 1..14: mol_type = other DNA
cttgaggaagttgt

SEQ ID NO: 886 - DNA, 16 bp, synthetic construct
  misc_feature 1..16: note = synthetic sequence
  source 1..16: mol_type = other DNA
aggaagttgtagcacg

SEQ ID NO: 887 - DNA, 15 bp, synthetic construct
  misc_feature 1..15: note = synthetic sequence
  source 1..15: mol_type = other DNA
ctactaaaattaatt

SEQ ID NO: 888 - DNA, 15 bp, synthetic construct
  misc_feature 1..15: note = synthetic sequence
  source 1..15: mol_type = other DNA
tactaaaattaattt

SEQ ID NO: 889 - DNA, 14 bp, synthetic construct
  misc_feature 1..14: note = synthetic sequence
  source 1..14: mol_type = other DNA
actaaaattaattt

SEQ ID NO: 890 - DNA, 16 bp, synthetic construct
  misc_feature 1..16: note = synthetic sequence
  source 1..16: mol_type = other DNA
aattaattttacacat

SEQ ID NO: 891 - DNA, 16 bp, synthetic construct
  misc_feature 1..16: note = synthetic sequence
  source 1..16: mol_type = other DNA
attttacacattaggg

SEQ ID NO: 892 - DNA, 15 bp, synthetic construct
  misc_feature 1..15: note = synthetic sequence
  source 1..15: mol_type = other DNA
tacacattagggctc

SEQ ID NO: 893 - DNA, 15 bp, synthetic construct
  misc_feature 1..15: note = synthetic sequence
  source 1..15: mol_type = other DNA
acattagggctcttc

SEQ ID NO: 894 - DNA, 15 bp, synthetic construct
  misc_feature 1..15: note = synthetic sequence
  source 1..15: mol_type = other DNA
tagggctcttccata

SEQ ID NO: 895 - DNA, 15 bp, synthetic construct
  misc_feature 1..15: note = synthetic sequence
  source 1..15: mol_type = other DNA
gctcttccatatagg

SEQ ID NO: 896 - DNA, 16 bp, synthetic construct
  misc_feature 1..16: note = synthetic sequence
  source 1..16: mol_type = other DNA
aaggctctccatctta

SEQ ID NO: 897 - DNA, 14 bp, synthetic construct
  misc_feature 1..14: note = synthetic sequence
  source 1..14: mol_type = other DNA
aaggctctccatct

SEQ ID NO: 898 - DNA, 16 bp, synthetic construct
  misc_feature 1..16: note = synthetic sequence
  source 1..16: mol_type = other DNA
gctctccatcttacct

SEQ ID NO: 899 - DNA, 16 bp, synthetic construct
  misc_feature 1..16: note = synthetic sequence
  source 1..16: mol_type = other DNA
tccatcttacctttcg

SEQ ID NO: 900 - DNA, 16 bp, synthetic construct
  misc_feature 1..16: note = synthetic sequence
  source 1..16: mol_type = other DNA
cctccctaatgttaca

SEQ ID NO: 901 - DNA, 16 bp, synthetic construct
  misc_feature 1..16: note = synthetic sequence
  source 1..16: mol_type = other DNA
ctccctaatgttacag

SEQ ID NO: 902 - DNA, 16 bp, synthetic construct
  misc_feature 1..16: note = synthetic sequence
  source 1..16: mol_type = other DNA
ctccctaatgttacag

SEQ ID NO: 903 - DNA, 16 bp, synthetic construct
  misc_feature 1..16: note = synthetic sequence
  source 1..16: mol_type = other DNA
taaaaccaacactacc

SEQ ID NO: 904 - DNA, 16 bp, synthetic construct
  misc_feature 1..16: note = synthetic sequence
  source 1..16: mol_type = other DNA
aaaccaacactaccac

SEQ ID NO: 905 - DNA, 16 bp, synthetic construct
  misc_feature 1..16: note = synthetic sequence
  source 1..16: mol_type = other DNA
aaaccaacactaccac

SEQ ID NO: 906 - DNA, 16 bp, synthetic construct
  misc_feature 1..16: note = synthetic sequence
  source 1..16: mol_type = other DNA
accaacactaccacat

SEQ ID NO: 907 - DNA, 16 bp, synthetic construct
  misc_feature 1..16: note = synthetic sequence
  source 1..16: mol_type = other DNA
caacactaccacatga

SEQ ID NO: 908 - DNA, 16 bp, synthetic construct
  misc_feature 1..16: note = synthetic sequence
  source 1..16: mol_type = other DNA
caacactaccacatga